European Patent Application EP 4 682 164 A1, published January 21, 2026. Title: New fusion protein for treating autoimmune diseases. Applicant: CUROGEN Technology Co., Ltd. Application KR PT24-5308, filed March 15, 2024. The sequence listing filed with the application follows.

SEQUENCE LISTING (115 sequences)

SEQ ID NO: 1 - protein, 931 aa, synthetic construct
  REGION 1..931: note = IL-17RA/RC-Fc-TNFR2 (T1T4-14)
LRLLDHRAPVCSQPGLNCTVKNSDCLDDSWIHPRNLTPSSPKDLQIQLHFAHTQQGDLVPVAHIEWTLQTDASILYLEGAELSVLQLDTNERLCVRFEFLSKLRHHHRRWRFTFSHFVVDPGQEYEVTVHHLPKPIPDGDPNHQSKNFLVPDCEHPRMKVTTPCMSSALPWLNVSADGDNVHLVLNVSEEQHFGLSLYWNQVQGPPKPRWHKNLTGPQIITLNHTDLVPCLCIQVWPLEPDSVRTNICPFREDPRAHQNLWQAARLRLLTLQSWLLDAPCSLPAEAALCWRAPGGDPCQPLVPPLSWENVTVDKVLEFPLLKGHPNLCVQVNSSEKLQLQECLWADSLGPLKDDVLLLETRGPQDNRSLCALEPSGCTSLPSKASTRAARLGEYLLQDLQSGQCLQLWDDDLGALWACPMDKYIHKTGIEGRMDRNTGRGGEEKKKEKEKEEQEERETKTPECPSHTQPLGVFLFPPKPKDTLMISRTPEVTCVVVDVSQEDPEVQFNWYVDGVEVHNAKTKPREEQFNSTYRVVSVLTVLHQDWLNGKEYKCKVSNKGLPSSIEKTISKAKGQPREPQVYTLPPSQEEMTKNQVSLTCLVKGFYPSDIAVEWESNGQPENNYKTTPPVLDSDGSFFLYSRLTVDKSRWQEGNVFSCSVMHEALHNHYTQKSLSLSLGKGGGGSGGGGSGGGGSLELPAQVAFTPYAPEPGSTCRLREYYDQTAQMCCAKCPPGQHAKVFCTKTSDTVCDSCEDSTYTQLWNWVPECLSCSSRCSSDQVETQACTREQNRICTCRPGWYCALSKQEGCRLCAPLSKCRPGFGVARPGTETSDVVCKPCAPGTFSNTTSSTDICRPHQICSVVAIPGNASMDAVCTSTSPTRSMAPGAVHLPQPVSTRSQHTQPTPGPSTAPSTSILLPMGPSPPAEGSTGD

SEQ ID NO: 2 - protein, 931 aa, synthetic construct
  REGION 1..931: note = IL-17RA/RC-Fc-TNFR2 (T1T4-05)
LRLLDHRALVCSQPGLNCTVKNSTCLDDSWIHPRNLTPSSPKDLQIQLHFAHTQQGDLFPVAHIEWTLQTDASILYLEGAELSVLQLNTNERLCVRFEFLSKLRHHHRRWRFTFSHFVVDPDQEYEVTVHHLPKPIPDGDPNHQSKNFLVPDCEHARMKVTTPCMSSALPWLNVSADGDNVHLVLNVSEEQHFGLSLYWNQVQGPPKPRWHKNLTGPQIITLNHTDLVPCLCIQVWPLEPDSVRTNICPFREDPRAHQNLWQAARLRLLTLQSWLLDAPCSLPAEAALCWRAPGGDPCQPLVPPLSWENVTVDKVLEFPLLKGHPNLCVQVNSSEKLQLQECLWADSLGPLKDDVLLLETRGPQDNRSLCALEPSGCTSLPSKASTRAARLGEYLLQDLQSGQCLQLWDDDLGALWACPMDKYIHKTGIEGRMDRNTGRGGEEKKKEKEKEEQEERETKTPECPSHTQPLGVFLFPPKPKDTLMISRTPEVTCVVVDVSQEDPEVQFNWYVDGVEVHNAKTKPREEQFNSTYRVVSVLTVLHQDWLNGKEYKCKVSNKGLPSSIEKTISKAKGQPREPQVYTLPPSQEEMTKNQVSLTCLVKGFYPSDIAVEWESNGQPENNYKTTPPVLDSDGSFFLYSRLTVDKSRWQEGNVFSCSVMHEALHNHYTQKSLSLSLGKGGGGSGGGGSGGGGSLELPAQVAFTPYAPEPGSTCRLREYYDQTAQMCCSKCSPGQHAKVFCTKTSDTVCDSCEDSTYTQLWNWVPECLSCGSRCSSDQVETQACTREQNRICTCRPGWYCALSKQEGCRLCAPLRKCRPGFGVARPGTETSDVVCKPCAPGTFSNTTSSTDICRPHQICNVVAIPGNASMDAVCTSTSPTRSMAPGAVHLPQPVSTRSQHTQPTPEPSTAPSTSFLLPMGPSPPAEGSTGD

SEQ ID NO: 3 - DNA, 2892 bp, synthetic construct
  misc_feature 1..2892: note = IL-17RA/RC-Fc-TNFR2 (T1T4-05)
  source 1..2892: mol_type = other DNA
atgggtgctgcgcgcagtccaccgagtgctgtgcccggtccattgctgggattgctgctccttcttcttggggtgcttgccccaggtggagcaagccttcggttgctcgaccacagggccttggtctgctcccaacctggcctgaattgtacagtcaagaactcaacgtgcttggatgattcatggattcatccacgaaacctcacgcctagcagtcctaaagatttgcaaattcaacttcatttcgcgcacacgcagcaaggagatttgttccctgttgctcatattgagtggactcttcaaacggacgcctcaattctgtacttggagggagcagaactgtccgttctgcagcttaatacaaacgaaaggctctgtgtcagattcgagttccttagtaaacttcgacatcatcacaggagatggcgatttacattctcccatttcgtggtcgatccggaccaagaatacgaagttacggtgcaccacctgccgaagccaatccccgacggggacccgaaccaccagtccaagaattttctcgttcccgactgtgagcacgcgaggatgaaagtgaccacaccttgcatgtcatcagccttgccttggttgaatgtcagcgctgatggagacaatgtgcatctcgtcctgaatgtgtccgaggaacaacattttggactgtctctgtactggaatcaggtacagggcccccctaaaccaaggtggcacaaaaatttgaccggaccgcaaatcatcacactcaatcatactgatcttgtgccttgtctgtgcattcaagtttggccactggagccagactctgtgagaactaatatctgcccttttcgggaggacccgagggcccatcagaatttgtggcaagctgcacgactgcggcttctgacgttgcaatcatggctgcttgacgcgccttgttcccttccagcagaggcagcgctctgctggagggctccaggaggtgacccctgccagccactcgtgccgccactgagttgggaaaatgtcactgtggataaggtccttgagtttccactgctgaagggacatccaaacctttgcgtccaagttaactcttcagagaagcttcagttgcaggagtgtttgtgggcggactctttgggccccctgaaggatgacgtcctccttctcgaaacgcgaggcccacaggataatcgcagcctttgcgcgctggagccaagtggatgcacatcattgccatccaaggcctctacccgggctgctcgactcggggagtatctgctgcaggatctgcagtctggacaatgcctccagctgtgggacgacgatctcggggctctctgggcctgcccaatggacaagtatatccataagaccggtatcgagggcaggatggaccgcaatactgggcggggcggggaggaaaagaaaaaggagaaggaaaaggaggaacaggaggaaagagagactaagaccccagaatgtcccagccatactcagcccctgggggtgttcctgtttccccctaaacctaaggataccctgatgatcagcaggacacccgaggtgacctgcgtggtcgtggatgtgagccaggaagatcccgaagtgcagttcaactggtacgtggatggcgtggaagtgcacaacgccaagaccaagcccagagaagagcagttcaactccacctacagagtggtgagcgtgctgaccgtgctgcaccaggactggctgaacggcaaggagtacaagtgcaaggtgtccaacaaaggcctgcccagctccatcgagaagaccatcagcaaagccaaaggccagcccagagaaccccaggtgtacaccctgcctcccagccaggaagagatgaccaagaaccaggtgtccctgacctgcctggtgaaaggcttctaccccagcgacatcgccgtggagtgggaaagcaacggccagcccgagaacaattacaagacaacccctcccgtgctggatagcgatggcagcttctttctgtacagcagactgaccgtggacaagagcagatggcaggaaggcaacgtgttcagctgcagcgtgatgcacgaagccctgcacaaccactacacccagaagagcctgtccctgagcctgggcaagggtggaggtggttctggaggtggaggatctggaggaggtggttctctcgagctgcccgcccaggtggcttttaccccttacgcccccgagcccggaagcacctgtagactgagagagtactacgaccagactgctcagatgtgctgctctaaatgctcccctggccagcacgccaaggtgttctgcaccaagacctccgacaccgtctgcgactcctgcgaggattctacctatacccagctgtggaattgggtgcctgagtgcctgtcctgcggctctagatgctcctctgatcaagtggaaacccaggcctgtaccagagagcagaaccggatctgtacatgtcggcctggttggtactgtgctctgtccaagcaagagggctgtcggctgtgcgctcctctgcggaagtgccgccctggcttcggcgtggccagaccaggcaccgagacatctgacgtggtgtgcaagccttgtgccccaggaaccttctccaacaccacctccagcacagatatctgcagacctcaccagatctgcaacgtggtcgccatccctggcaacgcctctatggacgcagtttgcacctctacaagccccaccagatccatggctccaggcgccgtgcacctgcctcagcctgtgtccacccggtctcagcacacccagcctacccccgaaccctctaccgccccttccacatccttcctgctgcctatgggccctagccctcctgccgaaggctccaccggcgactaa

SEQ ID NO: 4 - protein, 931 aa, synthetic construct
  REGION 1..931: note = IL-17RA/RC-Fc-TNFR2 (T1T4-06)
LRLLDHRAPVCSQPGLNCTVKNSDCLDDSWIHPRNLTPSSPKDLQIQLHFAHTQQGDLVPVAHIEWTLQTDASILYLEGAELSVLQLDTNERLCVRFEFLSKLRHHHRRWRFTFSHFVVDPGQEYEVTVHHLPKPIPDGDPNHQSKNFLVPDCEHARMKVTTPCMSSALPWLNVSADGDNVHLVLNVSEEQHFGLSLYWNQVQGPPKPRWHKNLTGPQIITLNHTDLVPCLCIQVWPLEPDSVRTNICPFREDPRAHQNLWQAARLRLLTLQSWLLDAPCSLPAEAALCWRAPGGDPCQPLVPPLSWENVTVDKVLEFPLLKGHPNLCVQVNSSEKLQLQECLWADSLGPLKDDVLLLETRGPQDNRSLCALEPSGCTSLPSKASTRAARLGEYLLQDLQSGQCLQLWDDDLGALWACPMDKYIHKTGIEGRMDRNTGRGGEEKKKEKEKEEQEERETKTPECPSHTQPLGVFLFPPKPKDTLMISRTPEVTCVVVDVSQEDPEVQFNWYVDGVEVHNAKTKPREEQFNSTYRVVSVLTVLHQDWLNGKEYKCKVSNKGLPSSIEKTISKAKGQPREPQVYTLPPSQEEMTKNQVSLTCLVKGFYPSDIAVEWESNGQPENNYKTTPPVLDSDGSFFLYSRLTVDKSRWQEGNVFSCSVMHEALHNHYTQKSLSLSLGKGGGGSGGGGSGGGGSLELPAQVAFTPYAPEPGSTCRLREYYDQTAQMCCSKCSPGQHAKVFCTKTSDTVCDSCEDSTYTQLWNWVPECLSCGSRCSSDQVETQACTREQNRICTCRPGWYCALSKQEGCRLCAPLRKCRPGFGVARPGTETSDVVCKPCAPGTFSNTTSSTDICRPHQICNVVAIPGNASMDAVCTSTSPTRSMAPGAVHLPQPVSTRSQHTQPTPEPSTAPSTSFLLPMGPSPPAEGSTGD

SEQ ID NO: 5 - DNA, 2892 bp, synthetic construct
  misc_feature 1..2892: note = IL-17RA/RC-Fc-TNFR2 (T1T4-06)
  source 1..2892: mol_type = other DNA
atgggtgctgcgcgcagtccaccgagtgctgtgcccggtccattgctgggattgctgctccttcttcttggggtgcttgccccaggtggagcaagccttcggttgctcgaccacagggcccccgtctgctcccaacctggcctgaattgtacagtcaagaactcagactgcttggatgattcatggattcatccacgaaacctcacgcctagcagtcctaaagatttgcaaattcaacttcatttcgcgcacacgcagcaaggagatttggtgcctgttgctcatattgagtggactcttcaaacggacgcctcaattctgtacttggagggagcagaactgtccgttctgcagcttgacacaaacgaaaggctctgtgtcagattcgagttccttagtaaacttcgacatcatcacaggagatggcgatttacattctcccatttcgtggtcgatccgggccaagaatacgaagttacggtgcaccacctgccgaagccaatccccgacggggacccgaaccaccagtccaagaattttctcgttcccgactgtgagcacgcgaggatgaaagtgaccacaccttgcatgtcatcagccttgccttggttgaatgtcagcgctgatggagacaatgtgcatctcgtcctgaatgtgtccgaggaacaacattttggactgtctctgtactggaatcaggtacagggcccccctaaaccaaggtggcacaaaaatttgaccggaccgcaaatcatcacactcaatcatactgatcttgtgccttgtctgtgcattcaagtttggccactggagccagactctgtgagaactaatatctgcccttttcgggaggacccgagggcccatcagaatttgtggcaagctgcacgactgcggcttctgacgttgcaatcatggctgcttgacgcgccttgttcccttccagcagaggcagcgctctgctggagggctccaggaggtgacccctgccagccactcgtgccgccactgagttgggaaaatgtcactgtggataaggtccttgagtttccactgctgaagggacatccaaacctttgcgtccaagttaactcttcagagaagcttcagttgcaggagtgtttgtgggcggactctttgggccccctgaaggatgacgtcctccttctcgaaacgcgaggcccacaggataatcgcagcctttgcgcgctggagccaagtggatgcacatcattgccatccaaggcctctacccgggctgctcgactcggggagtatctgctgcaggatctgcagtctggacaatgcctccagctgtgggacgacgatctcggggctctctgggcctgcccaatggacaagtatatccataagaccggtatcgagggcaggatggaccgcaatactgggcggggcggggaggaaaagaaaaaggagaaggaaaaggaggaacaggaggaaagagagactaagaccccagaatgtcccagccatactcagcccctgggggtgttcctgtttccccctaaacctaaggataccctgatgatcagcaggacacccgaggtgacctgcgtggtcgtggatgtgagccaggaagatcccgaagtgcagttcaactggtacgtggatggcgtggaagtgcacaacgccaagaccaagcccagagaagagcagttcaactccacctacagagtggtgagcgtgctgaccgtgctgcaccaggactggctgaacggcaaggagtacaagtgcaaggtgtccaacaaaggcctgcccagctccatcgagaagaccatcagcaaagccaaaggccagcccagagaaccccaggtgtacaccctgcctcccagccaggaagagatgaccaagaaccaggtgtccctgacctgcctggtgaaaggcttctaccccagcgacatcgccgtggagtgggaaagcaacggccagcccgagaacaattacaagacaacccctcccgtgctggatagcgatggcagcttctttctgtacagcagactgaccgtggacaagagcagatggcaggaaggcaacgtgttcagctgcagcgtgatgcacgaagccctgcacaaccactacacccagaagagcctgtccctgagcctgggcaagggtggaggtggttctggaggtggaggatctggaggaggtggttctctcgagctgcccgcccaggtggcttttaccccttacgcccccgagcccggaagcacctgtagactgagagagtactacgaccagactgctcagatgtgctgctctaaatgctcccctggccagcacgccaaggtgttctgcaccaagacctccgacaccgtctgcgactcctgcgaggattctacctatacccagctgtggaattgggtgcctgagtgcctgtcctgcggctctagatgctcctctgatcaagtggaaacccaggcctgtaccagagagcagaaccggatctgtacatgtcggcctggttggtactgtgctctgtccaagcaagagggctgtcggctgtgcgctcctctgcggaagtgccgccctggcttcggcgtggccagaccaggcaccgagacatctgacgtggtgtgcaagccttgtgccccaggaaccttctccaacaccacctccagcacagatatctgcagacctcaccagatctgcaacgtggtcgccatccctggcaacgcctctatggacgcagtttgcacctctacaagccccaccagatccatggctccaggcgccgtgcacctgcctcagcctgtgtccacccggtctcagcacacccagcctacccccgaaccctctaccgccccttccacatccttcctgctgcctatgggccctagccctcctgccgaaggctccaccggcgactaa

SEQ ID NO: 6 - protein, 931 aa, synthetic construct
  REGION 1..931: note = IL-17RA/RC-Fc-TNFR2 (T1T4-07)
LRLLDHRAPVCSQPGLNCTVKNSDCLDDSWIHPRNLTPSSPKDLQIQLHFAHTQQGDLVPVAHIEWTLQTDASILYLEGAELSVLQLDTNERLCVRFEFLSKLRHHHRRWRFTFSHFVVDPGQEYEVTVHHLPKPIPDGDPNHQSKNFLVPDCEHPRMKVTTPCMSSALPWLNVSADGDNVHLVLNVSEEQHFGLSLYWNQVQGPPKPRWHKNLTGPQIITLNHTDLVPCLCIQVWPLEPDSVRTNICPFREDPRAHQNLWQAARLRLLTLQSWLLDAPCSLPAEAALCWRAPGGDPCQPLVPPLSWENVTVDKVLEFPLLKGHPNLCVQVNSSEKLQLQECLWADSLGPLKDDVLLLETRGPQDNRSLCALEPSGCTSLPSKASTRAARLGEYLLQDLQSGQCLQLWDDDLGALWACPMDKYIHKTGIEGRMDRNTGRGGEEKKKEKEKEEQEERETKTPECPSHTQPLGVFLFPPKPKDTLMISRTPEVTCVVVDVSQEDPEVQFNWYVDGVEVHNAKTKPREEQFNSTYRVVSVLTVLHQDWLNGKEYKCKVSNKGLPSSIEKTISKAKGQPREPQVYTLPPSQEEMTKNQVSLTCLVKGFYPSDIAVEWESNGQPENNYKTTPPVLDSDGSFFLYSRLTVDKSRWQEGNVFSCSVMHEALHNHYTQKSLSLSLGKGGGGSGGGGSGGGGSLELPAQVAFTPYAPEPGSTCRLREYYDQTAQMCCSKCSPGQHAKVFCTKTSDTVCDSCEDSTYTQLWNWVPECLSCGSRCSSDQVETQACTREQNRICTCRPGWYCALSKQEGCRLCAPLRKCRPGFGVARPGTETSDVVCKPCAPGTFSNTTSSTDICRPHQICNVVAIPGNASMDAVCTSTSPTRSMAPGAVHLPQPVSTRSQHTQPTPEPSTAPSTSFLLPMGPSPPAEGSTGD

SEQ ID NO: 7 - DNA, 2892 bp, synthetic construct
  misc_feature 1..2892: note = IL-17RA/RC-Fc-TNFR2 (T1T4-07)
  source 1..2892: mol_type = other DNA
atgggtgctgcgcgcagtccaccgagtgctgtgcccggtccattgctgggattgctgctccttcttcttggggtgcttgccccaggtggagcaagccttcggttgctcgaccacagggcccccgtctgctcccaacctggcctgaattgtacagtcaagaactcagactgcttggatgattcatggattcatccacgaaacctcacgcctagcagtcctaaagatttgcaaattcaacttcatttcgcgcacacgcagcaaggagatttggtgcctgttgctcatattgagtggactcttcaaacggacgcctcaattctgtacttggagggagcagaactgtccgttctgcagcttgacacaaacgaaaggctctgtgtcagattcgagttccttagtaaacttcgacatcatcacaggagatggcgatttacattctcccatttcgtggtcgatccgggccaagaatacgaagttacggtgcaccacctgccgaagccaatccccgacggggacccgaaccaccagtccaagaattttctcgttcccgactgtgagcaccctaggatgaaagtgaccacaccttgcatgtcatcagccttgccttggttgaatgtcagcgctgatggagacaatgtgcatctcgtcctgaatgtgtccgaggaacaacattttggactgtctctgtactggaatcaggtacagggcccccctaaaccaaggtggcacaaaaatttgaccggaccgcaaatcatcacactcaatcatactgatcttgtgccttgtctgtgcattcaagtttggccactggagccagactctgtgagaactaatatctgcccttttcgggaggacccgagggcccatcagaatttgtggcaagctgcacgactgcggcttctgacgttgcaatcatggctgcttgacgcgccttgttcccttccagcagaggcagcgctctgctggagggctccaggaggtgacccctgccagccactcgtgccgccactgagttgggaaaatgtcactgtggataaggtccttgagtttccactgctgaagggacatccaaacctttgcgtccaagttaactcttcagagaagcttcagttgcaggagtgtttgtgggcggactctttgggccccctgaaggatgacgtcctccttctcgaaacgcgaggcccacaggataatcgcagcctttgcgcgctggagccaagtggatgcacatcattgccatccaaggcctctacccgggctgctcgactcggggagtatctgctgcaggatctgcagtctggacaatgcctccagctgtgggacgacgatctcggggctctctgggcctgcccaatggacaagtatatccataagaccggtatcgagggcaggatggaccgcaatactgggcggggcggggaggaaaagaaaaaggagaaggaaaaggaggaacaggaggaaagagagactaagaccccagaatgtcccagccatactcagcccctgggggtgttcctgtttccccctaaacctaaggataccctgatgatcagcaggacacccgaggtgacctgcgtggtcgtggatgtgagccaggaagatcccgaagtgcagttcaactggtacgtggatggcgtggaagtgcacaacgccaagaccaagcccagagaagagcagttcaactccacctacagagtggtgagcgtgctgaccgtgctgcaccaggactggctgaacggcaaggagtacaagtgcaaggtgtccaacaaaggcctgcccagctccatcgagaagaccatcagcaaagccaaaggccagcccagagaaccccaggtgtacaccctgcctcccagccaggaagagatgaccaagaaccaggtgtccctgacctgcctggtgaaaggcttctaccccagcgacatcgccgtggagtgggaaagcaacggccagcccgagaacaattacaagacaacccctcccgtgctggatagcgatggcagcttctttctgtacagcagactgaccgtggacaagagcagatggcaggaaggcaacgtgttcagctgcagcgtgatgcacgaagccctgcacaaccactacacccagaagagcctgtccctgagcctgggcaagggtggaggtggttctggaggtggaggatctggaggaggtggttctctcgagctgcccgcccaggtggcttttaccccttacgcccccgagcccggaagcacctgtagactgagagagtactacgaccagactgctcagatgtgctgctctaaatgctcccctggccagcacgccaaggtgttctgcaccaagacctccgacaccgtctgcgactcctgcgaggattctacctatacccagctgtggaattgggtgcctgagtgcctgtcctgcggctctagatgctcctctgatcaagtggaaacccaggcctgtaccagagagcagaaccggatctgtacatgtcggcctggttggtactgtgctctgtccaagcaagagggctgtcggctgtgcgctcctctgcggaagtgccgccctggcttcggcgtggccagaccaggcaccgagacatctgacgtggtgtgcaagccttgtgccccaggaaccttctccaacaccacctccagcacagatatctgcagacctcaccagatctgcaacgtggtcgccatccctggcaacgcctctatggacgcagtttgcacctctacaagccccaccagatccatggctccaggcgccgtgcacctgcctcagcctgtgtccacccggtctcagcacacccagcctacccccgaaccctctaccgccccttccacatccttcctgctgcctatgggccctagccctcctgccgaaggctccaccggcgactaa

SEQ ID NO: 8 - protein, 931 aa, synthetic construct
  REGION 1..931: note = IL-17RA/RC-Fc-TNFR2 (T1T4-08)
LRLLDHRAPVCSQPGLNCTVKNSDCLDDSWIHPRNLTPSSPKDLQIQLHFAHTQQGDLVPVAHIEWTLQTDASILYLEGAELSVLQLDTNERLCVRFEFLSKLRHHHRRWRFTFSHFVVDPGQEYEVTVHHLPKPIPDGDPNHQSKNFLVPDCEHPRMKVTTPCMSSALPWLNVSADGDNVHLVLNVSEEQHFGLSLYWNQVQGPPKPRWHKNLTGPQIITLNHTDLVPCLCIQVWPLEPDSVRTNICPFREDPRAHQNLWQAARLRLLTLQSWLLDAPCSLPAEAALCWRAPGGDPCQPLVPPLSWENVTVDKVLEFPLLKGHPNLCVQVNSSEKLQLQECLWADSLGPLKDDVLLLETRGPQDNRSLCALEPSGCTSLPSKASTRAARLGEYLLQDLQSGQCLQLWDDDLGALWACPMDKYIHKTGIEGRMDRNTGRGGEEKKKEKEKEEQEERETKTPECPSHTQPLGVFLFPPKPKDTLMISRTPEVTCVVVDVSQEDPEVQFNWYVDGVEVHNAKTKPREEQFNSTYRVVSVLTVLHQDWLNGKEYKCKVSNKGLPSSIEKTISKAKGQPREPQVYTLPPSQEEMTKNQVSLTCLVKGFYPSDIAVEWESNGQPENNYKTTPPVLDSDGSFFLYSRLTVDKSRWQEGNVFSCSVMHEALHNHYTQKSLSLSLGKGGGGSGGGGSGGGGSLELPAQVAFTPYAPEPGSTCRLREYYDQTAQMCCAKCSPGQHAKVFCTKTSDTVCDSCEDSTYTQLWNWVPECLSCGSRCSSDQVETQACTREQNRICTCRPGWYCALSKQEGCRLCAPLRKCRPGFGVARPGTETSDVVCKPCAPGTFSNTTSSTDICRPHQICNVVAIPGNASMDAVCTSTSPTRSMAPGAVHLPQPVSTRSQHTQPTPEPSTAPSTSFLLPMGPSPPAEGSTGD

SEQ ID NO: 9 - DNA, 2892 bp, synthetic construct
  misc_feature 1..2892: note = IL-17RA/RC-Fc-TNFR2 (T1T4-08)
  source 1..2892: mol_type = other DNA
atgggtgctgcgcgcagtccaccgagtgctgtgcccggtccattgctgggattgctgctccttcttcttggggtgcttgccccaggtggagcaagccttcggttgctcgaccacagggcccccgtctgctcccaacctggcctgaattgtacagtcaagaactcagactgcttggatgattcatggattcatccacgaaacctcacgcctagcagtcctaaagatttgcaaattcaacttcatttcgcgcacacgcagcaaggagatttggtgcctgttgctcatattgagtggactcttcaaacggacgcctcaattctgtacttggagggagcagaactgtccgttctgcagcttgacacaaacgaaaggctctgtgtcagattcgagttccttagtaaacttcgacatcatcacaggagatggcgatttacattctcccatttcgtggtcgatccgggccaagaatacgaagttacggtgcaccacctgccgaagccaatccccgacggggacccgaaccaccagtccaagaattttctcgttcccgactgtgagcaccctaggatgaaagtgaccacaccttgcatgtcatcagccttgccttggttgaatgtcagcgctgatggagacaatgtgcatctcgtcctgaatgtgtccgaggaacaacattttggactgtctctgtactggaatcaggtacagggcccccctaaaccaaggtggcacaaaaatttgaccggaccgcaaatcatcacactcaatcatactgatcttgtgccttgtctgtgcattcaagtttggccactggagccagactctgtgagaactaatatctgcccttttcgggaggacccgagggcccatcagaatttgtggcaagctgcacgactgcggcttctgacgttgcaatcatggctgcttgacgcgccttgttcccttccagcagaggcagcgctctgctggagggctccaggaggtgacccctgccagccactcgtgccgccactgagttgggaaaatgtcactgtggataaggtccttgagtttccactgctgaagggacatccaaacctttgcgtccaagttaactcttcagagaagcttcagttgcaggagtgtttgtgggcggactctttgggccccctgaaggatgacgtcctccttctcgaaacgcgaggcccacaggataatcgcagcctttgcgcgctggagccaagtggatgcacatcattgccatccaaggcctctacccgggctgctcgactcggggagtatctgctgcaggatctgcagtctggacaatgcctccagctgtgggacgacgatctcggggctctctgggcctgcccaatggacaagtatatccataagaccggtatcgagggcaggatggaccgcaatactgggcggggcggggaggaaaagaaaaaggagaaggaaaaggaggaacaggaggaaagagagactaagaccccagaatgtcccagccatactcagcccctgggggtgttcctgtttccccctaaacctaaggataccctgatgatcagcaggacacccgaggtgacctgcgtggtcgtggatgtgagccaggaagatcccgaagtgcagttcaactggtacgtggatggcgtggaagtgcacaacgccaagaccaagcccagagaagagcagttcaactccacctacagagtggtgagcgtgctgaccgtgctgcaccaggactggctgaacggcaaggagtacaagtgcaaggtgtccaacaaaggcctgcccagctccatcgagaagaccatcagcaaagccaaaggccagcccagagaaccccaggtgtacaccctgcctcccagccaggaagagatgaccaagaaccaggtgtccctgacctgcctggtgaaaggcttctaccccagcgacatcgccgtggagtgggaaagcaacggccagcccgagaacaattacaagacaacccctcccgtgctggatagcgatggcagcttctttctgtacagcagactgaccgtggacaagagcagatggcaggaaggcaacgtgttcagctgcagcgtgatgcacgaagccctgcacaaccactacacccagaagagcctgtccctgagcctgggcaagggtggaggtggttctggaggtggaggatctggaggaggtggttctctcgagctgcccgcccaggtggcttttaccccttacgcccccgagcccggaagcacctgtagactgagagagtactacgaccagactgctcagatgtgctgcgccaaatgctcccctggccagcacgccaaggtgttctgcaccaagacctccgacaccgtctgcgactcctgcgaggattctacctatacccagctgtggaattgggtgcctgagtgcctgtcctgcggctctagatgctcctctgatcaagtggaaacccaggcctgtaccagagagcagaaccggatctgtacatgtcggcctggttggtactgtgctctgtccaagcaagagggctgtcggctgtgcgctcctctgcggaagtgccgccctggcttcggcgtggccagaccaggcaccgagacatctgacgtggtgtgcaagccttgtgccccaggaaccttctccaacaccacctccagcacagatatctgcagacctcaccagatctgcaacgtggtcgccatccctggcaacgcctctatggacgcagtttgcacctctacaagccccaccagatccatggctccaggcgccgtgcacctgcctcagcctgtgtccacccggtctcagcacacccagcctacccccgaaccctctaccgccccttccacatccttcctgctgcctatgggccctagccctcctgccgaaggctccaccggcgactaa

SEQ ID NO: 10 - protein, 931 aa, synthetic construct
  REGION 1..931: note = IL-17RA/RC-Fc-TNFR2 (T1T4-09)
LRLLDHRAPVCSQPGLNCTVKNSDCLDDSWIHPRNLTPSSPKDLQIQLHFAHTQQGDLVPVAHIEWTLQTDASILYLEGAELSVLQLDTNERLCVRFEFLSKLRHHHRRWRFTFSHFVVDPGQEYEVTVHHLPKPIPDGDPNHQSKNFLVPDCEHPRMKVTTPCMSSALPWLNVSADGDNVHLVLNVSEEQHFGLSLYWNQVQGPPKPRWHKNLTGPQIITLNHTDLVPCLCIQVWPLEPDSVRTNICPFREDPRAHQNLWQAARLRLLTLQSWLLDAPCSLPAEAALCWRAPGGDPCQPLVPPLSWENVTVDKVLEFPLLKGHPNLCVQVNSSEKLQLQECLWADSLGPLKDDVLLLETRGPQDNRSLCALEPSGCTSLPSKASTRAARLGEYLLQDLQSGQCLQLWDDDLGALWACPMDKYIHKTGIEGRMDRNTGRGGEEKKKEKEKEEQEERETKTPECPSHTQPLGVFLFPPKPKDTLMISRTPEVTCVVVDVSQEDPEVQFNWYVDGVEVHNAKTKPREEQFNSTYRVVSVLTVLHQDWLNGKEYKCKVSNKGLPSSIEKTISKAKGQPREPQVYTLPPSQEEMTKNQVSLTCLVKGFYPSDIAVEWESNGQPENNYKTTPPVLDSDGSFFLYSRLTVDKSRWQEGNVFSCSVMHEALHNHYTQKSLSLSLGKGGGGSGGGGSGGGGSLELPAQVAFTPYAPEPGSTCRLREYYDQTAQMCCAKCPPGQHAKVFCTKTSDTVCDSCEDSTYTQLWNWVPECLSCGSRCSSDQVETQACTREQNRICTCRPGWYCALSKQEGCRLCAPLRKCRPGFGVARPGTETSDVVCKPCAPGTFSNTTSSTDICRPHQICNVVAIPGNASMDAVCTSTSPTRSMAPGAVHLPQPVSTRSQHTQPTPEPSTAPSTSFLLPMGPSPPAEGSTGD

SEQ ID NO: 11 - DNA, 2892 bp, synthetic construct
  misc_feature 1..2892: note = IL-17RA/RC-Fc-TNFR2 (T1T4-09)
  source 1..2892: mol_type = other DNA
atgggtgctgcgcgcagtccaccgagtgctgtgcccggtccattgctgggattgctgctccttcttcttggggtgcttgccccaggtggagcaagccttcggttgctcgaccacagggcccccgtctgctcccaacctggcctgaattgtacagtcaagaactcagactgcttggatgattcatggattcatccacgaaacctcacgcctagcagtcctaaagatttgcaaattcaacttcatttcgcgcacacgcagcaaggagatttggtgcctgttgctcatattgagtggactcttcaaacggacgcctcaattctgtacttggagggagcagaactgtccgttctgcagcttgacacaaacgaaaggctctgtgtcagattcgagttccttagtaaacttcgacatcatcacaggagatggcgatttacattctcccatttcgtggtcgatccgggccaagaatacgaagttacggtgcaccacctgccgaagccaatccccgacggggacccgaaccaccagtccaagaattttctcgttcccgactgtgagcaccctaggatgaaagtgaccacaccttgcatgtcatcagccttgccttggttgaatgtcagcgctgatggagacaatgtgcatctcgtcctgaatgtgtccgaggaacaacattttggactgtctctgtactggaatcaggtacagggcccccctaaaccaaggtggcacaaaaatttgaccggaccgcaaatcatcacactcaatcatactgatcttgtgccttgtctgtgcattcaagtttggccactggagccagactctgtgagaactaatatctgcccttttcgggaggacccgagggcccatcagaatttgtggcaagctgcacgactgcggcttctgacgttgcaatcatggctgcttgacgcgccttgttcccttccagcagaggcagcgctctgctggagggctccaggaggtgacccctgccagccactcgtgccgccactgagttgggaaaatgtcactgtggataaggtccttgagtttccactgctgaagggacatccaaacctttgcgtccaagttaactcttcagagaagcttcagttgcaggagtgtttgtgggcggactctttgggccccctgaaggatgacgtcctccttctcgaaacgcgaggcccacaggataatcgcagcctttgcgcgctggagccaagtggatgcacatcattgccatccaaggcctctacccgggctgctcgactcggggagtatctgctgcaggatctgcagtctggacaatgcctccagctgtgggacgacgatctcggggctctctgggcctgcccaatggacaagtatatccataagaccggtatcgagggcaggatggaccgcaatactgggcggggcggggaggaaaagaaaaaggagaaggaaaaggaggaacaggaggaaagagagactaagaccccagaatgtcccagccatactcagcccctgggggtgttcctgtttccccctaaacctaaggataccctgatgatcagcaggacacccgaggtgacctgcgtggtcgtggatgtgagccaggaagatcccgaagtgcagttcaactggtacgtggatggcgtggaagtgcacaacgccaagaccaagcccagagaagagcagttcaactccacctacagagtggtgagcgtgctgaccgtgctgcaccaggactggctgaacggcaaggagtacaagtgcaaggtgtccaacaaaggcctgcccagctccatcgagaagaccatcagcaaagccaaaggccagcccagagaaccccaggtgtacaccctgcctcccagccaggaagagatgaccaagaaccaggtgtccctgacctgcctggtgaaaggcttctaccccagcgacatcgccgtggagtgggaaagcaacggccagcccgagaacaattacaagacaacccctcccgtgctggatagcgatggcagcttctttctgtacagcagactgaccgtggacaagagcagatggcaggaaggcaacgtgttcagctgcagcgtgatgcacgaagccctgcacaaccactacacccagaagagcctgtccctgagcctgggcaagggtggaggtggttctggaggtggaggatctggaggaggtggttctctcgagctgcccgcccaggtggcttttaccccttacgcccccgagcccggaagcacctgtagactgagagagtactacgaccagactgctcagatgtgctgcgccaaatgccctcctggccagcacgccaaggtgttctgcaccaagacctccgacaccgtctgcgactcctgcgaggattctacctatacccagctgtggaattgggtgcctgagtgcctgtcctgcggctctagatgctcctctgatcaagtggaaacccaggcctgtaccagagagcagaaccggatctgtacatgtcggcctggttggtactgtgctctgtccaagcaagagggctgtcggctgtgcgctcctctgcggaagtgccgccctggcttcggcgtggccagaccaggcaccgagacatctgacgtggtgtgcaagccttgtgccccaggaaccttctccaacaccacctccagcacagatatctgcagacctcaccagatctgcaacgtggtcgccatccctggcaacgcctctatggacgcagtttgcacctctacaagccccaccagatccatggctccaggcgccgtgcacctgcctcagcctgtgtccacccggtctcagcacacccagcctacccccgaaccctctaccgccccttccacatccttcctgctgcctatgggccctagccctcctgccgaaggctccaccggcgactaa

SEQ ID NO: 12 - protein, 931 aa, synthetic construct
  REGION 1..931: note = IL-17RA/RC-Fc-TNFR2 (T1T4-10)
LRLLDHRAPVCSQPGLNCTVKNSDCLDDSWIHPRNLTPSSPKDLQIQLHFAHTQQGDLVPVAHIEWTLQTDASILYLEGAELSVLQLDTNERLCVRFEFLSKLRHHHRRWRFTFSHFVVDPGQEYEVTVHHLPKPIPDGDPNHQSKNFLVPDCEHPRMKVTTPCMSSALPWLNVSADGDNVHLVLNVSEEQHFGLSLYWNQVQGPPKPRWHKNLTGPQIITLNHTDLVPCLCIQVWPLEPDSVRTNICPFREDPRAHQNLWQAARLRLLTLQSWLLDAPCSLPAEAALCWRAPGGDPCQPLVPPLSWENVTVDKVLEFPLLKGHPNLCVQVNSSEKLQLQECLWADSLGPLKDDVLLLETRGPQDNRSLCALEPSGCTSLPSKASTRAARLGEYLLQDLQSGQCLQLWDDDLGALWACPMDKYIHKTGIEGRMDRNTGRGGEEKKKEKEKEEQEERETKTPECPSHTQPLGVFLFPPKPKDTLMISRTPEVTCVVVDVSQEDPEVQFNWYVDGVEVHNAKTKPREEQFNSTYRVVSVLTVLHQDWLNGKEYKCKVSNKGLPSSIEKTISKAKGQPREPQVYTLPPSQEEMTKNQVSLTCLVKGFYPSDIAVEWESNGQPENNYKTTPPVLDSDGSFFLYSRLTVDKSRWQEGNVFSCSVMHEALHNHYTQKSLSLSLGKGGGGSGGGGSGGGGSLELPAQVAFTPYAPEPGSTCRLREYYDQTAQMCCAKCPPGQHAKVFCTKTSDTVCDSCEDSTYTQLWNWVPECLSCGSRCSSDQVETQACTREQNRICTCRPGWYCALSKQEGCRLCAPLSKCRPGFGVARPGTETSDVVCKPCAPGTFSNTTSSTDICRPHQICNVVAIPGNASMDAVCTSTSPTRSMAPGAVHLPQPVSTRSQHTQPTPEPSTAPSTSFLLPMGPSPPAEGSTGD

SEQ ID NO: 13 - DNA, 2891 bp, synthetic construct
  misc_feature 1..2891: note = IL-17RA/RC-Fc-TNFR2 (T1T4-10)
  source 1..2891: mol_type = other DNA
atgggtgctgcgcgcagtccaccgagtgctgtgcccggtccattgctgggattgctgctccttcttcttggggtgcttgccccaggtggagcaagccttcggttgctcgaccacagggcccccgtctgctcccaacctggcctgaattgtacagtcaagaactcagactgcttggatgattcatggattcatccacgaaacctcacgcctagcagtcctaaagatttgcaaattcaacttcatttcgcgcacacgcagcaaggagatttggtgcctgttgctcatattgagtggactcttcaaacggacgcctcaattctgtacttggagggagcagaactgtccgttctgcagcttgacacaaacgaaaggctctgtgtcagattcgagttccttagtaaacttcgacatcatcacaggagatggcgatttacattctcccatttcgtggtcgatccgggccaagaatacgaagttacggtgcaccacctgccgaagccaatccccgacggggacccgaaccaccagtccaagaattttctcgttcccgactgtgagcaccctaggatgaaagtgaccacaccttgcatgtcatcagccttgccttggttgaatgtcagcgctgatggagacaatgtgcatctcgtcctgaatgtgtccgaggaacaacattttggactgtctctgtactggaatcaggtacagggcccccctaaaccaaggtggcacaaaaatttgaccggaccgcaaatcatcacactcaatcatactgatcttgtgccttgtctgtgcattcaagtttggccactggagccagactctgtgagaactaatatctgcccttttcgggaggacccgagggcccatcagaatttgtggcaagctgcacgactgcggcttctgacgttgcaatcatggctgcttgacgcgccttgttcccttccagcagaggcagcgctctgctggagggctccaggaggtgacccctgccagccactcgtgccgccactgagttgggaaaatgtcactgtggataaggtccttgagtttccactgctgaagggacatccaaacctttgcgtccaagttaactcttcagagaagcttcagttgcaggagtgtttgtgggcggactctttgggccccctgaaggatgacgtcctccttctcgaaacgcgaggcccacaggataatcgcagcctttgcgcgctggagccaagtggatgcacatcattgccatccaaggcctctacccgggctgctcgactcggggagtatctgctgcaggatctgcagtctggacaatgcctccagctgtgggacgacgatctcggggctctctgggcctgcccaatggacaagtatatccataagaccggtatcgagggcaggatggaccgcaatactgggcggggcggggaggaaaagaaaaaggagaaggaaaaggaggaacaggaggaaagagagactaagaccccagaatgtcccagccatactcagcccctgggggtgttcctgtttccccctaaacctaaggataccctgatgatcagcaggacacccgaggtgacctgcgtggtcgtggatgtgagccaggaagatcccgaagtgcagttcaactggtacgtggatggcgtggaagtgcacaacgccaagaccaagcccagagaagagcagttcaactccacctacagagtggtgagcgtgctgaccgtgctgcaccaggactggctgaacggcaaggagtacaagtgcaaggtgtccaacaaaggcctgcccagctccatcgagaagaccatcagcaaagccaaaggccagcccagagaaccccaggtgtacaccctgcctcccagccaggaagagatgaccaagaaccaggtgtccctgacctgcctggtgaaaggcttctaccccagcgacatcgccgtggagtgggaaagcaacggccagcccgagaacaattacaagacaacccctcccgtgctggatagcgatggcagcttctttctgtacagcagactgaccgtggacaagagcagatggcaggaaggcaacgtgttcagctgcagcgtgatgcacgaagccctgcacaaccactacacccagaagagcctgtccctgagcctgggcaagggtggaggtggttctggaggtggaggatctggaggaggtggttctctcgagctgcccgcccaggtggcttttaccccttacgcccccgagcccggaagcacctgtagactgagagagtactacgaccagactgctcagatgtgctgcgccaaatgccctcctggccagcacgccaaggtgttctgcaccaagacctccgacaccgtctgcgactcctgcgaggattctacctatacccagctgtggaattgggtgcctgagtgcctgtcctgcggctctagatgctcctctgatcaagtggaaacccaggcctgtaccagagagcagaaccggatctgtacatgtcggcctggttggtactgtgctctgtccaagcaagagggctgtcggctgtgcgctcctctgtccaagtgccgccctggcttcggcgtggccagaccaggcaccgagacatctgacgtggtgtgcaagccttgtgccccaggaaccttctccaacaccacctccagcacagatatctgcagacctcaccagatctgcaacgtggtcgccatccctggcaacgcctctatggacgcagtttgcacctctacaagccccaccagatccatggctccaggcgccgtgcacctgcctcagcctgtgtccacccggtctcagcacacccagcctacccccgaaccctctaccgccccttccacatccttcctgctgcctatgggccctagccctcctgccgaaggctccaccggcgacta

SEQ ID NO: 14 - protein, 931 aa, synthetic construct
  REGION 1..931: note = IL-17RA/RC-Fc-TNFR2 (T1T4-11)
LRLLDHRAPVCSQPGLNCTVKNSDCLDDSWIHPRNLTPSSPKDLQIQLHFAHTQQGDLVPVAHIEWTLQTDASILYLEGAELSVLQLDTNERLCVRFEFLSKLRHHHRRWRFTFSHFVVDPGQEYEVTVHHLPKPIPDGDPNHQSKNFLVPDCEHPRMKVTTPCMSSALPWLNVSADGDNVHLVLNVSEEQHFGLSLYWNQVQGPPKPRWHKNLTGPQIITLNHTDLVPCLCIQVWPLEPDSVRTNICPFREDPRAHQNLWQAARLRLLTLQSWLLDAPCSLPAEAALCWRAPGGDPCQPLVPPLSWENVTVDKVLEFPLLKGHPNLCVQVNSSEKLQLQECLWADSLGPLKDDVLLLETRGPQDNRSLCALEPSGCTSLPSKASTRAARLGEYLLQDLQSGQCLQLWDDDLGALWACPMDKYIHKTGIEGRMDRNTGRGGEEKKKEKEKEEQEERETKTPECPSHTQPLGVFLFPPKPKDTLMISRTPEVTCVVVDVSQEDPEVQFNWYVDGVEVHNAKTKPREEQFNSTYRVVSVLTVLHQDWLNGKEYKCKVSNKGLPSSIEKTISKAKGQPREPQVYTLPPSQEEMTKNQVSLTCLVKGFYPSDIAVEWESNGQPENNYKTTPPVLDSDGSFFLYSRLTVDKSRWQEGNVFSCSVMHEALHNHYTQKSLSLSLGKGGGGSGGGGSGGGGSLELPAQVAFTPYAPEPGSTCRLREYYDQTAQMCCAKCPPGQHAKVFCTKTSDTVCDSCEDSTYTQLWNWVPECLSCGSRCSSDQVETQACTREQNRICTCRPGWYCALSKQEGCRLCAPLSKCRPGFGVARPGTETSDVVCKPCAPGTFSNTTSSTDICRPHQICSVVAIPGNASMDAVCTSTSPTRSMAPGAVHLPQPVSTRSQHTQPTPEPSTAPSTSFLLPMGPSPPAEGSTGD

SEQ ID NO: 15 - DNA, 2892 bp, synthetic construct
  misc_feature 1..2892: note = IL-17RA/RC-Fc-TNFR2 (T1T4-11)
  source 1..2892: mol_type = other DNA
atgggtgctgcgcgcagtccaccgagtgctgtgcccggtccattgctgggattgctgctccttcttcttggggtgcttgccccaggtggagcaagccttcggttgctcgaccacagggcccccgtctgctcccaacctggcctgaattgtacagtcaagaactcagactgcttggatgattcatggattcatccacgaaacctcacgcctagcagtcctaaagatttgcaaattcaacttcatttcgcgcacacgcagcaaggagatttggtgcctgttgctcatattgagtggactcttcaaacggacgcctcaattctgtacttggagggagcagaactgtccgttctgcagcttgacacaaacgaaaggctctgtgtcagattcgagttccttagtaaacttcgacatcatcacaggagatggcgatttacattctcccatttcgtggtcgatccgggccaagaatacgaagttacggtgcaccacctgccgaagccaatccccgacggggacccgaaccaccagtccaagaattttctcgttcccgactgtgagcaccctaggatgaaagtgaccacaccttgcatgtcatcagccttgccttggttgaatgtcagcgctgatggagacaatgtgcatctcgtcctgaatgtgtccgaggaacaacattttggactgtctctgtactggaatcaggtacagggcccccctaaaccaaggtggcacaaaaatttgaccggaccgcaaatcatcacactcaatcatactgatcttgtgccttgtctgtgcattcaagtttggccactggagccagactctgtgagaactaatatctgcccttttcgggaggacccgagggcccatcagaatttgtggcaagctgcacgactgcggcttctgacgttgcaatcatggctgcttgacgcgccttgttcccttccagcagaggcagcgctctgctggagggctccaggaggtgacccctgccagccactcgtgccgccactgagttgggaaaatgtcactgtggataaggtccttgagtttccactgctgaagggacatccaaacctttgcgtccaagttaactcttcagagaagcttcagttgcaggagtgtttgtgggcggactctttgggccccctgaaggatgacgtcctccttctcgaaacgcgaggcccacaggataatcgcagcctttgcgcgctggagccaagtggatgcacatcattgccatccaaggcctctacccgggctgctcgactcggggagtatctgctgcaggatctgcagtctggacaatgcctccagctgtgggacgacgatctcggggctctctgggcctgcccaatggacaagtatatccataagaccggtatcgagggcaggatggaccgcaatactgggcggggcggggaggaaaagaaaaaggagaaggaaaaggaggaacaggaggaaagagagactaagaccccagaatgtcccagccatactcagcccctgggggtgttcctgtttccccctaaacctaaggataccctgatgatcagcaggacacccgaggtgacctgcgtggtcgtggatgtgagccaggaagatcccgaagtgcagttcaactggtacgtggatggcgtggaagtgcacaacgccaagaccaagcccagagaagagcagttcaactccacctacagagtggtgagcgtgctgaccgtgctgcaccaggactggctgaacggcaaggagtacaagtgcaaggtgtccaacaaaggcctgcccagctccatcgagaagaccatcagcaaagccaaaggccagcccagagaaccccaggtgtacaccctgcctcccagccaggaagagatgaccaagaaccaggtgtccctgacctgcctggtgaaaggcttctaccccagcgacatcgccgtggagtgggaaagcaacggccagcccgagaacaattacaagacaacccctcccgtgctggatagcgatggcagcttctttctgtacagcagactgaccgtggacaagagcagatggcaggaaggcaacgtgttcagctgcagcgtgatgcacgaagccctgcacaaccactacacccagaagagcctgtccctgagcctgggcaagggtggaggtggttctggaggtggaggatctggaggaggtggttctctcgagctgcccgcccaggtggcttttaccccttacgcccccgagcccggaagcacctgtagactgagagagtactacgaccagactgctcagatgtgctgcgccaaatgccctcctggccagcacgccaaggtgttctgcaccaagacctccgacaccgtctgcgactcctgcgaggattctacctatacccagctgtggaattgggtgcctgagtgcctgtcctgcggctctagatgctcctctgatcaagtggaaacccaggcctgtaccagagagcagaaccggatctgtacatgtcggcctggttggtactgtgctctgtccaagcaagagggctgtcggctgtgcgctcctctgtccaagtgccgccctggcttcggcgtggccagaccaggcaccgagacatctgacgtggtgtgcaagccttgtgccccaggaaccttctccaacaccacctccagcacagatatctgcagacctcaccagatctgctccgtggtcgccatccctggcaacgcctctatggacgcagtttgcacctctacaagccccaccagatccatggctccaggcgccgtgcacctgcctcagcctgtgtccacccggtctcagcacacccagcctacccccgaaccctctaccgccccttccacatccttcctgctgcctatgggccctagccctcctgccgaaggctccaccggcgactaa

SEQ ID NO: 16 - protein, 931 aa, synthetic construct
  REGION 1..931: note = IL-17RA/RC-Fc-TNFR2 (T1T4-12)
LRLLDHRAPVCSQPGLNCTVKNSDCLDDSWIHPRNLTPSSPKDLQIQLHFAHTQQGDLVPVAHIEWTLQTDASILYLEGAELSVLQLDTNERLCVRFEFLSKLRHHHRRWRFTFSHFVVDPGQEYEVTVHHLPKPIPDGDPNHQSKNFLVPDCEHPRMKVTTPCMSSALPWLNVSADGDNVHLVLNVSEEQHFGLSLYWNQVQGPPKPRWHKNLTGPQIITLNHTDLVPCLCIQVWPLEPDSVRTNICPFREDPRAHQNLWQAARLRLLTLQSWLLDAPCSLPAEAALCWRAPGGDPCQPLVPPLSWENVTVDKVLEFPLLKGHPNLCVQVNSSEKLQLQECLWADSLGPLKDDVLLLETRGPQDNRSLCALEPSGCTSLPSKASTRAARLGEYLLQDLQSGQCLQLWDDDLGALWACPMDKYIHKTGIEGRMDRNTGRGGEEKKKEKEKEEQEERETKTPECPSHTQPLGVFLFPPKPKDTLMISRTPEVTCVVVDVSQEDPEVQFNWYVDGVEVHNAKTKPREEQFNSTYRVVSVLTVLHQDWLNGKEYKCKVSNKGLPSSIEKTISKAKGQPREPQVYTLPPSQEEMTKNQVSLTCLVKGFYPSDIAVEWESNGQPENNYKTTPPVLDSDGSFFLYSRLTVDKSRWQEGNVFSCSVMHEALHNHYTQKSLSLSLGKGGGGSGGGGSGGGGSLELPAQVAFTPYAPEPGSTCRLREYYDQTAQMCCAKCPPGQHAKVFCTKTSDTVCDSCEDSTYTQLWNWVPECLSCGSRCSSDQVETQACTREQNRICTCRPGWYCALSKQEGCRLCAPLSKCRPGFGVARPGTETSDVVCKPCAPGTFSNTTSSTDICRPHQICSVVAIPGNASMDAVCTSTSPTRSMAPGAVHLPQPVSTRSQHTQPTPGPSTAPSTSFLLPMGPSPPAEGSTGD

SEQ ID NO: 17 - DNA, 2892 bp, synthetic construct
  misc_feature 1..2892: note = IL-17RA/RC-Fc-TNFR2 (T1T4-12)
  source 1..2892: mol_type = other DNA
atgggtgctgcgcgcagtccaccgagtgctgtgcccggtccattgctgggattgctgctccttcttcttggggtgcttgccccaggtggagcaagccttcggttgctcgaccacagggcccccgtctgctcccaacctggcctgaattgtacagtcaagaactcagactgcttggatgattcatggattcatccacgaaacctcacgcctagcagtcctaaagatttgcaaattcaacttcatttcgcgcacacgcagcaaggagatttggtgcctgttgctcatattgagtggactcttcaaacggacgcctcaattctgtacttggagggagcagaactgtccgttctgcagcttgacacaaacgaaaggctctgtgtcagattcgagttccttagtaaacttcgacatcatcacaggagatggcgatttacattctcccatttcgtggtcgatccgggccaagaatacgaagttacggtgcaccacctgccgaagccaatccccgacggggacccgaaccaccagtccaagaattttctcgttcccgactgtgagcaccctaggatgaaagtgaccacaccttgcatgtcatcagccttgccttggttgaatgtcagcgctgatggagacaatgtgcatctcgtcctgaatgtgtccgaggaacaacattttggactgtctctgtactggaatcaggtacagggcccccctaaaccaaggtggcacaaaaatttgaccggaccgcaaatcatcacactcaatcatactgatcttgtgccttgtctgtgcattcaagtttggccactggagccagactctgtgagaactaatatctgcccttttcgggaggacccgagggcccatcagaatttgtggcaagctgcacgactgcggcttctgacgttgcaatcatggctgcttgacgcgccttgttcccttccagcagaggcagcgctctgctggagggctccaggaggtgacccctgccagccactcgtgccgccactgagttgggaaaatgtcactgtggataaggtccttgagtttccactgctgaagggacatccaaacctttgcgtccaagttaactcttcagagaagcttcagttgcaggagtgtttgtgggcggactctttgggccccctgaaggatgacgtcctccttctcgaaacgcgaggcccacaggataatcgcagcctttgcgcgctggagccaagtggatgcacatcattgccatccaaggcctctacccgggctgctcgactcggggagtatctgctgcaggatctgcagtctggacaatgcctccagctgtgggacgacgatctcggggctctctgggcctgcccaatggacaagtatatccataagaccggtatcgagggcaggatggaccgcaatactgggcggggcggggaggaaaagaaaaaggagaaggaaaaggaggaacaggaggaaagagagactaagaccccagaatgtcccagccatactcagcccctgggggtgttcctgtttccccctaaacctaaggataccctgatgatcagcaggacacccgaggtgacctgcgtggtcgtggatgtgagccaggaagatcccgaagtgcagttcaactggtacgtggatggcgtggaagtgcacaacgccaagaccaagcccagagaagagcagttcaactccacctacagagtggtgagcgtgctgaccgtgctgcaccaggactggctgaacggcaaggagtacaagtgcaaggtgtccaacaaaggcctgcccagctccatcgagaagaccatcagcaaagccaaaggccagcccagagaaccccaggtgtacaccctgcctcccagccaggaagagatgaccaagaaccaggtgtccctgacctgcctggtgaaaggcttctaccccagcgacatcgccgtggagtgggaaagcaacggccagcccgagaacaattacaagacaacccctcccgtgctggatagcgatggcagcttctttctgtacagcagactgaccgtggacaagagcagatggcaggaaggcaacgtgttcagctgcagcgtgatgcacgaagccctgcacaaccactacacccagaagagcctgtccctgagcctgggcaagggtggaggtggttctggaggtggaggatctggaggaggtggttctctcgagctgcccgcccaggtggcttttaccccttacgcccccgagcccggaagcacctgtagactgagagagtactacgaccagactgctcagatgtgctgcgccaaatgccctcctggccagcacgccaaggtgttctgcaccaagacctccgacaccgtctgcgactcctgcgaggattctacctatacccagctgtggaattgggtgcctgagtgcctgtcctgcggctctagatgctcctctgatcaagtggaaacccaggcctgtaccagagagcagaaccggatctgtacatgtcggcctggttggtactgtgctctgtccaagcaagagggctgtcggctgtgcgctcctctgtccaagtgccgccctggcttcggcgtggccagaccaggcaccgagacatctgacgtggtgtgcaagccttgtgccccaggaaccttctccaacaccacctccagcacagatatctgcagacctcaccagatctgctccgtggtcgccatccctggcaacgcctctatggacgcagtttgcacctctacaagccccaccagatccatggctccaggcgccgtgcacctgcctcagcctgtgtccacccggtctcagcacacccagcctacccccggcccctctaccgccccttccacatccttcctgctgcctatgggccctagccctcctgccgaaggctccaccggcgactaa

SEQ ID NO: 18 - protein, 931 aa, synthetic construct
  REGION 1..931: note = IL-17RA/RC-Fc-TNFR2 (T1T4-13)
LRLLDHRAPVCSQPGLNCTVKNSDCLDDSWIHPRNLTPSSPKDLQIQLHFAHTQQGDLVPVAHIEWTLQTDASILYLEGAELSVLQLDTNERLCVRFEFLSKLRHHHRRWRFTFSHFVVDPGQEYEVTVHHLPKPIPDGDPNHQSKNFLVPDCEHPRMKVTTPCMSSALPWLNVSADGDNVHLVLNVSEEQHFGLSLYWNQVQGPPKPRWHKNLTGPQIITLNHTDLVPCLCIQVWPLEPDSVRTNICPFREDPRAHQNLWQAARLRLLTLQSWLLDAPCSLPAEAALCWRAPGGDPCQPLVPPLSWENVTVDKVLEFPLLKGHPNLCVQVNSSEKLQLQECLWADSLGPLKDDVLLLETRGPQDNRSLCALEPSGCTSLPSKASTRAARLGEYLLQDLQSGQCLQLWDDDLGALWACPMDKYIHKTGIEGRMDRNTGRGGEEKKKEKEKEEQEERETKTPECPSHTQPLGVFLFPPKPKDTLMISRTPEVTCVVVDVSQEDPEVQFNWYVDGVEVHNAKTKPREEQFNSTYRVVSVLTVLHQDWLNGKEYKCKVSNKGLPSSIEKTISKAKGQPREPQVYTLPPSQEEMTKNQVSLTCLVKGFYPSDIAVEWESNGQPENNYKTTPPVLDSDGSFFLYSRLTVDKSRWQEGNVFSCSVMHEALHNHYTQKSLSLSLGKGGGGSGGGGSGGGGSLELPAQVAFTPYAPEPGSTCRLREYYDQTAQMCCAKCPPGQHAKVFCTKTSDTVCDSCEDSTYTQLWNWVPECLSCGSRCSSDQVETQACTREQNRICTCRPGWYCALSKQEGCRLCAPLSKCRPGFGVARPGTETSDVVCKPCAPGTFSNTTSSTDICRPHQICSVVAIPGNASMDAVCTSTSPTRSMAPGAVHLPQPVSTRSQHTQPTPGPSTAPSTSILLPMGPSPPAEGSTGD

SEQ ID NO: 19 - DNA, 2892 bp, synthetic construct
  misc_feature 1..2892: note = IL-17RA/RC-Fc-TNFR2 (T1T4-13)
  source 1..2892: mol_type = other DNA
atgggtgctgcgcgcagtccaccgagtgctgtgcccggtccattgctgggattgctgctccttcttcttggggtgcttgccccaggtggagcaagccttcggttgctcgaccacagggcccccgtctgctcccaacctggcctgaattgtacagtcaagaactcagactgcttggatgattcatggattcatccacgaaacctcacgcctagcagtcctaaagatttgcaaattcaacttcatttcgcgcacacgcagcaaggagatttggtgcctgttgctcatattgagtggactcttcaaacggacgcctcaattctgtacttggagggagcagaactgtccgttctgcagcttgacacaaacgaaaggctctgtgtcagattcgagttccttagtaaacttcgacatcatcacaggagatggcgatttacattctcccatttcgtggtcgatccgggccaagaatacgaagttacggtgcaccacctgccgaagccaatccccgacggggacccgaaccaccagtccaagaattttctcgttcccgactgtgagcaccctaggatgaaagtgaccacaccttgcatgtcatcagccttgccttggttgaatgtcagcgctgatggagacaatgtgcatctcgtcctgaatgtgtccgaggaacaacattttggactgtctctgtactggaatcaggtacagggcccccctaaaccaaggtggcacaaaaatttgaccggaccgcaaatcatcacactcaatcatactgatcttgtgccttgtctgtgcattcaagtttggccactggagccagactctgtgagaactaatatctgcccttttcgggaggacccgagggcccatcagaatttgtggcaagctgcacgactgcggcttctgacgttgcaatcatggctgcttgacgcgccttgttcccttccagcagaggcagcgctctgctggagggctccaggaggtgacccctgccagccactcgtgccgccactgagttgggaaaatgtcactgtggataaggtccttgagtttccactgctgaagggacatccaaacctttgcgtccaagttaactcttcagagaagcttcagttgcaggagtgtttgtgggcggactctttgggccccctgaaggatgacgtcctccttctcgaaacgcgaggcccacaggataatcgcagcctttgcgcgctggagccaagtggatgcacatcattgccatccaaggcctctacccgggctgctcgactcggggagtatctgctgcaggatctgcagtctggacaatgcctccagctgtgggacgacgatctcggggctctctgggcctgcccaatggacaagtatatccataagaccggtatcgagggcaggatggaccgcaatactgggcggggcggggaggaaaagaaaaaggagaaggaaaaggaggaacaggaggaaagagagactaagaccccagaatgtcccagccatactcagcccctgggggtgttcctgtttccccctaaacctaaggataccctgatgatcagcaggacacccgaggtgacctgcgtggtcgtggatgtgagccaggaagatcccgaagtgcagttcaactggtacgtggatggcgtggaagtgcacaacgccaagaccaagcccagagaagagcagttcaactccacctacagagtggtgagcgtgctgaccgtgctgcaccaggactggctgaacggcaaggagtacaagtgcaaggtgtccaacaaaggcctgcccagctccatcgagaagaccatcagcaaagccaaaggccagcccagagaaccccaggtgtacaccctgcctcccagccaggaagagatgaccaagaaccaggtgtccctgacctgcctggtgaaaggcttctaccccagcgacatcgccgtggagtgggaaagcaacggccagcccgagaacaattacaagacaacccctcccgtgctggatagcgatggcagcttctttctgtacagcagactgaccgtggacaagagcagatggcaggaaggcaacgtgttcagctgcagcgtgatgcacgaagccctgcacaaccactacacccagaagagcctgtccctgagcctgggcaagggtggaggtggttctggaggtggaggatctggaggaggtggttctctcgagctgcccgcccaggtggcttttaccccttacgcccccgagcccggaagcacctgtagactgagagagtactacgaccagactgctcagatgtgctgcgccaaatgccctcctggccagcacgccaaggtgttctgcaccaagacctccgacaccgtctgcgactcctgcgaggattctacctatacccagctgtggaattgggtgcctgagtgcctgtcctgcggctctagatgctcctctgatcaagtggaaacccaggcctgtaccagagagcagaaccggatctgtacatgtcggcctggttggtactgtgctctgtccaagcaagagggctgtcggctgtgcgctcctctgtccaagtgccgccctggcttcggcgtggccagaccaggcaccgagacatctgacgtggtgtgcaagccttgtgccccaggaaccttctccaacaccacctccagcacagatatctgcagacctcaccagatctgctccgtggtcgccatccctggcaacgcctctatggacgcagtttgcacctctacaagccccaccagatccatggctccaggcgccgtgcacctgcctcagcctgtgtccacccggtctcagcacacccagcctacccccggcccctctaccgccccttccacatccatcctgctgcctatgggccctagccctcctgccgaaggctccaccggcgactaa

SEQ ID NO: 20 - protein, 931 aa, synthetic construct; identical to SEQ ID NO: 1
  REGION 1..931: note = IL-17RA/RC-Fc-TNFR2 (T1T4-14)

SEQ ID NO: 21 - DNA, 2892 bp, synthetic construct
  misc_feature 1..2892: note = IL-17RA/RC-Fc-TNFR2 (T1T4-14)
  source 1..2892: mol_type = other DNA
atgggtgctgcgcgcagtccaccgagtgctgtgcccggtccattgctgggattgctgctccttcttcttggggtgcttgccccaggtggagcaagccttcggttgctcgaccacagggcccccgtctgctcccaacctggcctgaattgtacagtcaagaactcagactgcttggatgattcatggattcatccacgaaacctcacgcctagcagtcctaaagatttgcaaattcaacttcatttcgcgcacacgcagcaaggagatttggtgcctgttgctcatattgagtggactcttcaaacggacgcctcaattctgtacttggagggagcagaactgtccgttctgcagcttgacacaaacgaaaggctctgtgtcagattcgagttccttagtaaacttcgacatcatcacaggagatggcgatttacattctcccatttcgtggtcgatccgggccaagaatacgaagttacggtgcaccacctgccgaagccaatccccgacggggacccgaaccaccagtccaagaattttctcgttcccgactgtgagcaccctaggatgaaagtgaccacaccttgcatgtcatcagccttgccttggttgaatgtcagcgctgatggagacaatgtgcatctcgtcctgaatgtgtccgaggaacaacattttggactgtctctgtactggaatcaggtacagggcccccctaaaccaaggtggcacaaaaatttgaccggaccgcaaatcatcacactcaatcatactgatcttgtgccttgtctgtgcattcaagtttggccactggagccagactctgtgagaactaatatctgcccttttcgggaggacccgagggcccatcagaatttgtggcaagctgcacgactgcggcttctgacgttgcaatcatggctgcttgacgcgccttgttcccttccagcagaggcagcgctctgctggagggctccaggaggtgacccctgccagccactcgtgccgccactgagttgggaaaatgtcactgtggataaggtccttgagtttccactgctgaagggacatccaaacctttgcgtccaagttaactcttcagagaagcttcagttgcaggagtgtttgtgggcggactctttgggccccctgaaggatgacgtcctccttctcgaaacgcgaggcccacaggataatcgcagcctttgcgcgctggagccaagtggatgcacatcattgccatccaaggcctctacccgggctgctcgactcggggagtatctgctgcaggatctgcagtctggacaatgcctccagctgtgggacgacgatctcggggctctctgggcctgcccaatggacaagtatatccataagaccggtatcgagggcaggatggaccgcaatactgggcggggcggggaggaaaagaaaaaggagaaggaaaaggaggaacaggaggaaagagagactaagaccccagaatgtcccagccatactcagcccctgggggtgttcctgtttccccctaaacctaaggataccctgatgatcagcaggacacccgaggtgacctgcgtggtcgtggatgtgagccaggaagatcccgaagtgcagttcaactggtacgtggatggcgtggaagtgcacaacgccaagaccaagcccagagaagagcagttcaactccacctacagagtggtgagcgtgctgaccgtgctgcaccaggactggctgaacggcaaggagtacaagtgcaaggtgtccaacaaaggcctgcccagctccatcgagaagaccatcagcaaagccaaaggccagcccagagaaccccaggtgtacaccctgcctcccagccaggaagagatgaccaagaaccaggtgtccctgacctgcctggtgaaaggcttctaccccagcgacatcgccgtggagtgggaaagcaacggccagcccgagaacaattacaagacaacccctcccgtgctggatagcgatggcagcttctttctgtacagcagactgaccgtggacaagagcagatggcaggaaggcaacgtgttcagctgcagcgtgatgcacgaagccctgcacaaccactacacccagaagagcctgtccctgagcctgggcaagggtggaggtggttctggaggtggaggatctggaggaggtggttctctcgagctgcccgcccaggtggcttttaccccttacgcccccgagcccggaagcacctgtagactgagagagtactacgaccagactgctcagatgtgctgcgccaaatgccctcctggccagcacgccaaggtgttctgcaccaagacctccgacaccgtctgcgactcctgcgaggattctacctatacccagctgtggaattgggtgcctgagtgcctgtcctgcagctctagatgctcctctgatcaagtggaaacccaggcctgtaccagagagcagaaccggatctgtacatgtcggcctggttggtactgtgctctgtccaagcaagagggctgtcggctgtgcgctcctctgtccaagtgccgccctggcttcggcgtggccagaccaggcaccgagacatctgacgtggtgtgcaagccttgtgccccaggaaccttctccaacaccacctccagcacagatatctgcagacctcaccagatctgctccgtggtcgccatccctggcaacgcctctatggacgcagtttgcacctctacaagccccaccagatccatggctccaggcgccgtgcacctgcctcagcctgtgtccacccggtctcagcacacccagcctacccccggcccctctaccgccccttccacatccatcctgctgcctatgggccctagccctcctgccgaaggctccaccggcgactaa

SEQ ID NO: 22 - protein, 931 aa, synthetic construct
  REGION 1..931: note = IL-17RA/RC-Fc-TNFR2 (T1T4-30)
LRLLDHRAPVCSQPGLNCTVKNSDCLDDSWIHPRNLTPSSPKDLQIQLHFAHTQQGDLVPVAHIEWTLQTDASILYLEGAELSVLQLDTNERLCVRFEFLSKLRHHHRRWRFTFSHFVVDPGQEYEVTVHHLPKPIPDGDPNHQSKNFLVPDCEHPRMKVTTPCMSSALPWLNVSADGDNVHLVLNVSEEQHFGLSLYWNQVQGPPKPRWHKNLTGPQIITLNHTDLVPCLCIQVWPLEPDSVRTNICPFREDPRAHQNLWQAARLRLLTLQSWLLDAPCSLPAEAALCWRAPGGDPCQPLVPPLSWENVTVDKVLEFPLLKGHPNLCVQVNSSEKLQLQECLWADSLGPLKDDVLLLETRGPQDNRSLCALEPSGCTSLPSKASTRAARLGEYLLQDLQSGQCLQLWDDDLGALWACPMDKYIHKTGIEGRMDRNTGRGGEEKKKEKEKEEQEERETKTPECPSHTQPLGVFLFPPKPKDTLMISRTPEVTCVVVDVSQEDPEVQFNWYVDGVEVHNAKTKPREEQFNSTYRVVSVLTVLHQDWLNGKEYKCKVSNKGLPSSIEKTISKAKGQPREPQVYTLPPSQEEMTKNQVSLTCLVKGFYPSDIAVEWESNGQPENNYKTTPPVLDSDGSFFLYSRLTVDKSRWQEGNVFSCSVMHEALHNHYTQKSLSLSLGKGGGGSGGGGSGGGGSLELPAQVAFTPYAPEPGSTCRLREYYDQTAQMCCSKCSPGQHAKVFCTKTSDTVCDSCEDSTYTQLWNWVPECLSCSSRCSSDQVETQACTREQNRICTCRPGWYCALSKQEGCRLCAPLRKCRPGFGVARPGTETSDVVCKPCAPGTFSNTTSSTDICRPHQICNVVAIPGNASMDAVCTSTSPTRSMAPGAVHLPQPVSTRSQHTQPTPEPSTAPSTSFLLPMGPSPPAEGSTGD

SEQ ID NO: 23 - DNA, 2892 bp, synthetic construct
  misc_feature 1..2892: note = IL-17RA/RC-Fc-TNFR2 (T1T4-30)
  source 1..2892: mol_type = other DNA
atgggtgctgcgcgcagtccaccgagtgctgtgcccggtccattgctgggattgctgctccttcttcttggggtgcttgccccaggtggagcaagccttcggttgctcgaccacagggcccccgtctgctcccaacctggcctgaattgtacagtcaagaactcagactgcttggatgattcatggattcatccacgaaacctcacgcctagcagtcctaaagatttgcaaattcaacttcatttcgcgcacacgcagcaaggagatttggtgcctgttgctcatattgagtggactcttcaaacggacgcctcaattctgtacttggagggagcagaactgtccgttctgcagcttgacacaaacgaaaggctctgtgtcagattcgagttccttagtaaacttcgacatcatcacaggagatggcgatttacattctcccatttcgtggtcgatccgggccaagaatacgaagttacggtgcaccacctgccgaagccaatccccgacggggacccgaaccaccagtccaagaattttctcgttcccgactgtgagcaccctaggatgaaagtgaccacaccttgcatgtcatcagccttgccttggttgaatgtcagcgctgatggagacaatgtgcatctcgtcctgaatgtgtccgaggaacaacattttggactgtctctgtactggaatcaggtacagggcccccctaaaccaaggtggcacaaaaatttgaccggaccgcaaatcatcacactcaatcatactgatcttgtgccttgtctgtgcattcaagtttggccactggagccagactctgtgagaactaatatctgcccttttcgggaggacccgagggcccatcagaatttgtggcaagctgcacgactgcggcttctgacgttgcaatcatggctgcttgacgcgccttgttcccttccagcagaggcagcgctctgctggagggctccaggaggtgacccctgccagccactcgtgccgccactgagttgggaaaatgtcactgtggataaggtccttgagtttccactgctgaagggacatccaaacctttgcgtccaagttaactcttcagagaagcttcagttgcaggagtgtttgtgggcggactctttgggccccctgaaggatgacgtcctccttctcgaaacgcgaggcccacaggataatcgcagcctttgcgcgctggagccaagtggatgcacatcattgccatccaaggcctctacccgggctgctcgactcggggagtatctgctgcaggatctgcagtctggacaatgcctccagctgtgggacgacgatctcggggctctctgggcctgcccaatggacaagtatatccataagaccggtatcgagggcaggatggaccgcaatactgggcggggcggggaggaaaagaaaaaggagaaggaaaaggaggaacaggaggaaagagagactaagaccccagaatgtcccagccatactcagcccctgggggtgttcctgtttccccctaaacctaaggataccctgatgatcagcaggacacccgaggtgacctgcgtggtcgtggatgtgagccaggaagatcccgaagtgcagttcaactggtacgtggatggcgtggaagtgcacaacgccaagaccaagcccagagaagagcagttcaactccacctacagagtggtgagcgtgctgaccgtgctgcaccaggactggctgaacggcaaggagtacaagtgcaaggtgtccaacaaaggcctgcccagctccatcgagaagaccatcagcaaagccaaaggccagcccagagaaccccaggtgtacaccctgcctcccagccaggaagagatgaccaagaaccaggtgtccctgacctgcctggtgaaaggcttctaccccagcgacatcgccgtggagtgggaaagcaacggccagcccgagaacaattacaagacaacccctcccgtgctggatagcgatggcagcttctttctgtacagcagactgaccgtggacaagagcagatggcaggaaggcaacgtgttcagctgcagcgtgatgcacgaagccctgcacaaccactacacccagaagagcctgtccctgagcctgggcaagggtggaggtggttctggaggtggaggatctggaggaggtggttctctcgagctgcccgcccaggtggcttttaccccttacgcccccgagcccggaagcacctgtagactgagagagtactacgaccagactgctcagatgtgctgctctaaatgctcccctggccagcacgccaaggtgttctgcaccaagacctccgacaccgtctgcgactcctgcgaggattctacctatacccagctgtggaattgggtgcctgagtgcctgtcctgcagctctagatgctcctctgatcaagtggaaacccaggcctgtaccagagagcagaaccggatctgtacatgtcggcctggttggtactgtgctctgtccaagcaagagggctgtcggctgtgcgctcctctgcggaagtgccgccctggcttcggcgtggccagaccaggcaccgagacatctgacgtggtgtgcaagccttgtgccccaggaaccttctccaacaccacctccagcacagatatctgcagacctcaccagatctgcaacgtggtcgccatccctggcaacgcctctatggacgcagtttgcacctctacaagccccaccagatccatggctccaggcgccgtgcacctgcctcagcctgtgtccacccggtctcagcacacccagcctacccccgaaccctctaccgccccttccacatccttcctgctgcctatgggccctagccctcctgccgaaggctccaccggcgactaa

SEQ ID NO: 24 - protein, 931 aa, synthetic construct
  REGION 1..931: note = IL-17RA/RC-Fc-TNFR2 (T1T4-31)
LRLLDHRAPVCSQPGLNCTVKNSDCLDDSWIHPRNLTPSSPKDLQIQLHFAHTQQGDLVPVAHIEWTLQTDASILYLEGAELSVLQLDTNERLCVRFEFLSKLRHHHRRWRFTFSHFVVDPGQEYEVTVHHLPKPIPDGDPNHQSKNFLVPDCEHPRMKVTTPCMSSALPWLNVSADGDNVHLVLNVSEEQHFGLSLYWNQVQGPPKPRWHKNLTGPQIITLNHTDLVPCLCIQVWPLEPDSVRTNICPFREDPRAHQNLWQAARLRLLTLQSWLLDAPCSLPAEAALCWRAPGGDPCQPLVPPLSWENVTVDKVLEFPLLKGHPNLCVQVNSSEKLQLQECLWADSLGPLKDDVLLLETRGPQDNRSLCALEPSGCTSLPSKASTRAARLGEYLLQDLQSGQCLQLWDDDLGALWACPMDKYIHKTGIEGRMDRNTGRGGEEKKKEKEKEEQEERETKTPECPSHTQPLGVFLFPPKPKDTLYITREPEVTCVVVDVSQEDPEVQFNWYVDGVEVHNAKTKPREEQFNSTYRVVSVLTVLHQDWLNGKEYKCKVSNKGLPSSIEKTISKAKGQPREPQVYTLPPSQEEMTKNQVSLTCLVKGFYPSDIAVEWESNGQPENNYKTTPPVLDSDGSFFLYSRLTVDKSRWQEGNVFSCSVMHEALHNHYTQKSLSLSLGKGGGGSGGGGSGGGGSLELPAQVAFTPYAPEPGSTCRLREYYDQTAQMCCAKCPPGQHAKVFCTKTSDTVCDSCEDSTYTQLWNWVPECLSCSSRCSSDQVETQACTREQNRICTCRPGWYCALSKQEGCRLCAPLSKCRPGFGVARPGTETSDVVCKPCAPGTFSNTTSSTDICRPHQICSVVAIPGNASMDAVCTSTSPTRSMAPGAVHLPQPVSTRSQHTQPTPGPSTAPSTSILLPMGPSPPAEGSTGD

SEQ ID NO: 25 - DNA, 2892 bp, synthetic construct
  misc_feature 1..2892: note = IL-17RA/RC-Fc-TNFR2 (T1T4-31)
  source 1..2892: mol_type = other DNA
atgggtgctgcgcgcagtccaccgagtgctgtgcccggtccattgctgggattgctgctccttcttcttggggtgcttgccccaggtggagcaagccttcggttgctcgaccacagggcccccgtctgctcccaacctggcctgaattgtacagtcaagaactcagactgcttggatgattcatggattcatccacgaaacctcacgcctagcagtcctaaagatttgcaaattcaacttcatttcgcgcacacgcagcaaggagatttggtgcctgttgctcatattgagtggactcttcaaacggacgcctcaattctgtacttggagggagcagaactgtccgttctgcagcttgacacaaacgaaaggctctgtgtcagattcgagttccttagtaaacttcgacatcatcacaggagatggcgatttacattctcccatttcgtggtcgatccgggccaagaatacgaagttacggtgcaccacctgccgaagccaatccccgacggggacccgaaccaccagtccaagaattttctcgttcccgactgtgagcaccctaggatgaaagtgaccacaccttgcatgtcatcagccttgccttggttgaatgtcagcgctgatggagacaatgtgcatctcgtcctgaatgtgtccgaggaacaacattttggactgtctctgtactggaatcaggtacagggcccccctaaaccaaggtggcacaaaaatttgaccggaccgcaaatcatcacactcaatcatactgatcttgtgccttgtctgtgcattcaagtttggccactggagccagactctgtgagaactaatatctgcccttttcgggaggacccgagggcccatcagaatttgtggcaagctgcacgactgcggcttctgacgttgcaatcatggctgcttgacgcgccttgttcccttccagcagaggcagcgctctgctggagggctccaggaggtgacccctgccagccactcgtgccgccactgagttgggaaaatgtcactgtggataaggtccttgagtttccactgctgaagggacatccaaacctttgcgtccaagttaactcttcagagaagcttcagttgcaggagtgtttgtgggcggactctttgggccccctgaaggatgacgtcctccttctcgaaacgcgaggcccacaggataatcgcagcctttgcgcgctggagccaagtggatgcacatcattgccatccaaggcctctacccgggctgctcgactcggggagtatctgctgcaggatctgcagtctggacaatgcctccagctgtgggacgacgatctcggggctctctgggcctgcccaatggacaagtatatccataagaccggtatcgagggcaggatggaccgcaatactgggcggggcggggaggaaaagaaaaaggagaaggaaaaggaggaacaggaggaaagagagactaagaccccagaatgtcccagccatactcagcccctgggggtgttcctgtttccccctaaacctaaggataccctgtacatcaccagggagcccgaggtgacctgcgtggtcgtggatgtgagccaggaagatcccgaagtgcagttcaactggtacgtggatggcgtggaagtgcacaacgccaagaccaagcccagagaagagcagttcaactccacctacagagtggtgagcgtgctgaccgtgctgcaccaggactggctgaacggcaaggagtacaagtgcaaggtgtccaacaaaggcctgcccagctccatcgagaagaccatcagcaaagccaaaggccagcccagagaaccccaggtgtacaccctgcctcccagccaggaagagatgaccaagaaccaggtgtccctgacctgcctggtgaaaggcttctaccccagcgacatcgccgtggagtgggaaagcaacggccagcccgagaacaattacaagacaacccctcccgtgctggatagcgatggcagcttctttctgtacagcagactgaccgtggacaagagcagatggcaggaaggcaacgtgttcagctgcagcgtgatgcacgaagccctgcacaaccactacacccagaagagcctgtccctgagcctgggcaagggtggaggtggttctggaggtggaggatctggaggaggtggttctctcgagctgcccgcccaggtggcttttaccccttacgcccccgagcccggaagcacctgtagactgagagagtactacgaccagactgctcagatgtgctgcgccaaatgccctcctggccagcacgccaaggtgttctgcaccaagacctccgacaccgtctgcgactcctgcgaggattctacctatacccagctgtggaattgggtgcctgagtgcctgtcctgcagctctagatgctcctctgatcaagtggaaacccaggcctgtaccagagagcagaaccggatctgtacatgtcggcctggttggtactgtgctctgtccaagcaagagggctgtcggctgtgcgctcctctgtccaagtgccgccctggcttcggcgtggccagaccaggcaccgagacatctgacgtggtgtgcaagccttgtgccccaggaaccttctccaacaccacctccagcacagatatctgcagacctcaccagatctgctccgtggtcgccatccctggcaacgcctctatggacgcagtttgcacctctacaagccccaccagatccatggctccaggcgccgtgcacctgcctcagcctgtgtccacccggtctcagcacacccagcctacccccggcccctctaccgccccttccacatccatcctgctgcctatgggccctagccctcctgccgaaggctccaccggcgactaa

SEQ ID NO: 26 - protein, 931 aa, synthetic construct
  REGION 1..931: note = IL-17RA/RC-Fc-TNFR2 (T1T4-32)
LRLLDHRAPVCSQPGLNCTVKNSDCLDDSWIHPRNLTPSSPKDLQIQLHFAHTQQGDLVPVAHIEWTLQTDASILYLEGAELSVLQLDTNERLCVRFEFLSKLRHHHRRWRFTFSHFVVDPGQEYEVTVHHLPKPIPDGDPNHQSKNFLVPDCEHPRMKVTTPCMSSALPWLNVSADGDNVHLVLNVSEEQHFGLSLYWNQVQGPPKPRWHKNLTGPQIITLNHTDLVPCLCIQVWPLEPDSVRTNICPFREDPRAHQNLWQAARLRLLTLQSWLLDAPCSLPAEAALCWRAPGGDPCQPLVPPLSWENVTVDKVLEFPLLKGHPNLCVQVNSSEKLQLQECLWADSLGPLKDDVLLLETRGPQDNRSLCALEPSGCTSLPSKASTRAARLGEYLLQDLQSGQCLQLWDDDLGALWACPMDKYIHKTGIEGRMDRNTGRGGEEKKKEKEKEEQEERETKTPECPSHTQPLGVFLFPPKPKDTLMISRTPEVTCVVVDVSQEDPEVQFNWYVDGVEVHNAKTKPREEQFNSTYRVVSVLTVLHQDWLNGKEYKCKVSNKGLPSSIEKTISKAKGQPREPQVYTLPPSQEEMTKNQVSLTCLVKGFYPSDIAVEWESNGQPENNYKTTPPVLDSDGSFFLYSRLTVDKSRWQEGNVFSCSVMHEALKFHYTQKSLSLSLGKGGGGSGGGGSGGGGSLELPAQVAFTPYAPEPGSTCRLREYYDQTAQMCCAKCPPGQHAKVFCTKTSDTVCDSCEDSTYTQLWNWVPECLSCSSRCSSDQVETQACTREQNRICTCRPGWYCALSKQEGCRLCAPLSKCRPGFGVARPGTETSDVVCKPCAPGTFSNTTSSTDICRPHQICSVVAIPGNASMDAVCTSTSPTRSMAPGAVHLPQPVSTRSQHTQPTPGPSTAPSTSILLPMGPSPPAEGSTGD

SEQ ID NO: 27 - DNA, 2892 bp, synthetic construct
  misc_feature 1..2892: note = IL-17RA/RC-Fc-TNFR2 (T1T4-32)
  source 1..2892: mol_type = other DNA
atgggtgctgcgcgcagtccaccgagtgctgtgcccggtccattgctgggattgctgctccttcttcttggggtgcttgccccaggtggagcaagccttcggttgctcgaccacagggcccccgtctgctcccaacctggcctgaattgtacagtcaagaactcagactgcttggatgattcatggattcatccacgaaacctcacgcctagcagtcctaaagatttgcaaattcaacttcatttcgcgcacacgcagcaaggagatttggtgcctgttgctcatattgagtggactcttcaaacggacgcctcaattctgtacttggagggagcagaactgtccgttctgcagcttgacacaaacgaaaggctctgtgtcagattcgagttccttagtaaacttcgacatcatcacaggagatggcgatttacattctcccatttcgtggtcgatccgggccaagaatacgaagttacggtgcaccacctgccgaagccaatccccgacggggacccgaaccaccagtccaagaattttctcgttcccgactgtgagcaccctaggatgaaagtgaccacaccttgcatgtcatcagccttgccttggttgaatgtcagcgctgatggagacaatgtgcatctcgtcctgaatgtgtccgaggaacaacattttggactgtctctgtactggaatcaggtacagggcccccctaaaccaaggtggcacaaaaatttgaccggaccgcaaatcatcacactcaatcatactgatcttgtgccttgtctgtgcattcaagtttggccactggagccagactctgtgagaactaatatctgcccttttcgggaggacccgagggcccatcagaatttgtggcaagctgcacgactgcggcttctgacgttgcaatcatggctgcttgacgcgccttgttcccttccagcagaggcagcgctctgctggagggctccaggaggtgacccctgccagccactcgtgccgccactgagttgggaaaatgtcactgtggataaggtccttgagtttccactgctgaagggacatccaaacctttgcgtccaagttaactcttcagagaagcttcagttgcaggagtgtttgtgggcggactctttgggccccctgaaggatgacgtcctccttctcgaaacgcgaggcccacaggataatcgcagcctttgcgcgctggagccaagtggatgcacatcattgccatccaaggcctctacccgggctgctcgactcggggagtatctgctgcaggatctgcagtctggacaatgcctccagctgtgggacgacgatctcggggctctctgggcctgcccaatggacaagtatatccataagaccggtatcgagggcaggatggaccgcaatactgggcggggcggggaggaaaagaaaaaggagaaggaaaaggaggaacaggaggaaagagagactaagaccccagaatgtcccagccatactcagcccctgggggtgttcctgtttccccctaaacctaaggataccctgatgatcagcaggacacccgaggtgacctgcgtggtcgtggatgtgagccaggaagatcccgaagtgcagttcaactggtacgtggatggcgtggaagtgcacaacgccaagaccaagcccagagaagagcagttcaactccacctacagagtggtgagcgtgctgaccgtgctgcaccaggactggctgaacggcaaggagtacaagtgcaaggtgtccaacaaaggcctgcccagctccatcgagaagaccatcagcaaagccaaaggccagcccagagaaccccaggtgtacaccctgcctcccagccaggaagagatgaccaagaaccaggtgtccctgacctgcctggtgaaaggcttctaccccagcgacatcgccgtggagtgggaaagcaacggccagcccgagaacaattacaagacaacccctcccgtgctggatagcgatggcagcttctttctgtacagcagactgaccgtggacaagagcagatggcaggaaggcaacgtgttcagctgcagcgtgatgcacgaagccctgaagttccactacacccagaagagcctgtccctgagcctgggcaagggtggaggtggttctggaggtggaggatctggaggaggtggttctctcgagctgcccgcccaggtggcttttaccccttacgcccccgagcccggaagcacctgtagactgagagagtactacgaccagactgctcagatgtgctgcgccaaatgccctcctggccagcacgccaaggtgttctgcaccaagacctccgacaccgtctgcgactcctgcgaggattctacctatacccagctgtggaattgggtgcctgagtgcctgtcctgcagctctagatgctcctctgatcaagtggaaacccaggcctgtaccagagagcagaaccggatctgtacatgtcggcctggttggtactgtgctctgtccaagcaagagggctgtcggctgtgcgctcctctgtccaagtgccgccctggcttcggcgtggccagaccaggcaccgagacatctgacgtggtgtgcaagccttgtgccccaggaaccttctccaacaccacctccagcacagatatctgcagacctcaccagatctgctccgtggtcgccatccctggcaacgcctctatggacgcagtttgcacctctacaagccccaccagatccatggctccaggcgccgtgcacctgcctcagcctgtgtccacccggtctcagcacacccagcctacccccggcccctctaccgccccttccacatccatcctgctgcctatgggccctagccctcctgccgaaggctccaccggcgactaa

SEQ ID NO: 28 - protein, 897 aa, synthetic construct
  REGION 1..897: note = IL-17RA/RC-Fc-TNFR2 (T1T4-33)
LRLLDHRAPVCSQPGLNCTVKNSDCLDDSWIHPRNLTPSSPKDLQIQLHFAHTQQGDLVPVAHIEWTLQTDASILYLEGAELSVLQLDTNERLCVRFEFLSKLRHHHRRWRFTFSHFVVDPGQEYEVTVHHLPKPIPDGDPNHQSKNFLVPDCEHPRMKVTTPCMSSALPWLNVSADGDNVHLVLNVSEEQHFGLSLYWNQVQGPPKPRWHKNLTGPQIITLNHTDLVPCLCIQVWPLEPDSVRTNICPFREDPRAHQNLWQAARLRLLTLQSWLLDAPCSLPAEAALCWRAPGGDPCQPLVPPLSWENVTVDKVLEFPLLKGHPNLCVQVNSSEKLQLQECLWADSLGPLKDDVLLLETRGPQDNRSLCALEPSGCTSLPSKASTRAARLGEYLLQDLQSGQCLQLWDDDLGALWACPMDKYIHKTGIEGRMDRNTGRGGEEKKKEKEKEEQEERETKTPECPSHTQPLGVFLFPPKPKDTLMISRTPEVTCVVVDVSQEDPEVQFNWYVDGVEVHNAKTKPREEQFNSTYRVVSVLTVLHQDWLNGKEYKCKVSNKGLPSSIEKTISKAKGQPREPQVYTLPPSQEEMTKNQVSLTCLVKGFYPSDIAVEWESNGQPENNYKTTPPVLDSDGSFFLYSRLTVDKSRWQEGNVFSCSVMHEALHNHYTQKSLSLSLGKGGGGSGGGGSGGGGSLELPAQVAFTPYAPEPGSTCRLREYYDQTAQMCCAKCPPGQHAKVFCTKTSDTVCDSCEDSTYTQLWNWVPECLSCSSRCSSDQVETQACTREQNRICTCRPGWYCALSKQEGCRLCAPLSKCRPGFGVARPGTETSDVVCKPCAPGTFSNTTSSTDICRPHQICSVVAIPGNASMDAVCTSTSPTRSMAPGAVHLPQPVSTR

SEQ ID NO: 29 - DNA, 2790 bp, synthetic construct
  misc_feature 1..2790: note = IL-17RA/RC-Fc-TNFR2 (T1T4-33)
  source 1..2790: mol_type = other DNA
atgggtgctgcgcgcagtccaccgagtgctgtgcccggtccattgctgggattgctgctccttcttcttggggtgcttgccccaggtggagcaagccttcggttgctcgaccacagggcccccgtctgctcccaacctggcctgaattgtacagtcaagaactcagactgcttggatgattcatggattcatccacgaaacctcacgcctagcagtcctaaagatttgcaaattcaacttcatttcgcgcacacgcagcaaggagatttggtgcctgttgctcatattgagtggactcttcaaacggacgcctcaattctgtacttggagggagcagaactgtccgttctgcagcttgacacaaacgaaaggctctgtgtcagattcgagttccttagtaaacttcgacatcatcacaggagatggcgatttacattctcccatttcgtggtcgatccgggccaagaatacgaagttacggtgcaccacctgccgaagccaatccccgacggggacccgaaccaccagtccaagaattttctcgttcccgactgtgagcaccctaggatgaaagtgaccacaccttgcatgtcatcagccttgccttggttgaatgtcagcgctgatggagacaatgtgcatctcgtcctgaatgtgtccgaggaacaacattttggactgtctctgtactggaatcaggtacagggcccccctaaaccaaggtggcacaaaaatttgaccggaccgcaaatcatcacactcaatcatactgatcttgtgccttgtctgtgcattcaagtttggccactggagccagactctgtgagaactaatatctgcccttttcgggaggacccgagggcccatcagaatttgtggcaagctgcacgactgcggcttctgacgttgcaatcatggctgcttgacgcgccttgttcccttccagcagaggcagcgctctgctggagggctccaggaggtgacccctgccagccactcgtgccgccactgagttgggaaaatgtcactgtggataaggtccttgagtttccactgctgaagggacatccaaacctttgcgtccaagttaactcttcagagaagcttcagttgcaggagtgtttgtgggcggactctttgggccccctgaaggatgacgtcctccttctcgaaacgcgaggcccacaggataatcgcagcctttgcgcgctggagccaagtggatgcacatcattgccatccaaggcctctacccgggctgctcgactcggggagtatctgctgcaggatctgcagtctggacaatgcctccagctgtgggacgacgatctcggggctctctgggcctgcccaatggacaagtatatccataagaccggtatcgagggcaggatggaccgcaatactgggcggggcggggaggaaaagaaaaaggagaaggaaaaggaggaacaggaggaaagagagactaagaccccagaatgtcccagccatactcagcccctgggggtgttcctgtttccccctaaacctaaggataccctgatgatcagcaggacacccgaggtgacctgcgtggtcgtggatgtgagccaggaagatcccgaagtgcagttcaactggtacgtggatggcgtggaagtgcacaacgccaagaccaagcccagagaagagcagttcaactccacctacagagtggtgagcgtgctgaccgtgctgcaccaggactggctgaacggcaaggagtacaagtgcaaggtgtccaacaaaggcctgcccagctccatcgagaagaccatcagcaaagccaaaggccagcccagagaaccccaggtgtacaccctgcctcccagccaggaagagatgaccaagaaccaggtgtccctgacctgcctggtgaaaggcttctaccccagcgacatcgccgtggagtgggaaagcaacggccagcccgagaacaattacaagacaacccctcccgtgctggatagcgatggcagcttctttctgtacagcagactgaccgtggacaagagcagatggcaggaaggcaacgtgttcagctgcagcgtgatgcacgaagccctgcacaaccactacacccagaagagcctgtccctgagcctgggcaagggtggaggtggttctggaggtggaggatctggaggaggtggttctctcgagctgcccgcccaggtggcttttaccccttacgcccccgagcccggaagcacctgtagactgagagagtactacgaccagactgctcagatgtgctgcgccaaatgccctcctggccagcacgccaaggtgttctgcaccaagacctccgacaccgtctgcgactcctgcgaggattctacctatacccagctgtggaattgggtgcctgagtgcctgtcctgcagctctagatgctcctctgatcaagtggaaacccaggcctgtaccagagagcagaaccggatctgtacatgtcggcctggttggtactgtgctctgtccaagcaagagggctgtcggctgtgcgctcctctgtccaagtgccgccctggcttcggcgtggccagaccaggcaccgagacatctgacgtggtgtgcaagccttgtgccccaggaaccttctccaacaccacctccagcacagatatctgcagacctcaccagatctgctccgtggtcgccatccctggcaacgcctctatggacgcagtttgcacctctacaagccccaccagatccatggctccaggcgccgtgcacctgcctcagcctgtgtccacccggtaa

SEQ ID NO: 30 - protein, 1144 aa, synthetic construct
  REGION 1..1144: note = IL-17RA/RC-Fc-TNFR2 (T1T4-34)
LRLLDHRAPVCSQPGLNCTVKNSDCLDDSWIHPRNLTPSSPKDLQIQLHFAHTQQGDLVPVAHIEWTLQTDASILYLEGAELSVLQLDTNERLCVRFEFLSKLRHHHRRWRFTFSHFVVDPGQEYEVTVHHLPKPIPDGDPNHQSKNFLVPDCEHPRMKVTTPCMSSALPWLNVSADGDNVHLVLNVSEEQHFGLSLYWNQVQGPPKPRWHKNLTGPQIITLNHTDLVPCLCIQVWPLEPDSVRTNICPFREDPRAHQNLWQAARLRLLTLQSWLLDAPCSLPAEAALCWRAPGGDPCQPLVPPLSWENVTVDKVLEFPLLKGHPNLCVQVNSSEKLQLQECLWADSLGPLKDDVLLLETRGPQDNRSLCALEPSGCTSLPSKASTRAARLGEYLLQDLQSGQCLQLWDDDLGALWACPMDKYIHKTGIEGRMDRNTGRGGEEKKKEKEKEEQEERETKTPECPSHTQPLGVFLFPPKPKDTLMISRTPEVTCVVVDVSQEDPEVQFNWYVDGVEVHNAKTKPREEQFNSTYRVVSVLTVLHQDWLNGKEYKCKVSNKGLPSSIEKTISKAKGQPREPQVYTLPPSQEEMTKNQVSLTCLVKGFYPSDIAVEWESNGQPENNYKTTPPVLDSDGSFFLYSRLTVDKSRWQEGNVFSCSVMHEALHNHYTQKSLSLSLGKGGGGSGGGGSGGGGSLELPAQVAFTPYAPEPGSTCRLREYYDQTAQMCCAKCPPGQHAKVFCTKTSDTVCDSCEDSTYTQLWNWVPECLSCSSRCSSDQVETQACTREQNRICTCRPGWYCALSKQEGCRLCAPLSKCRPGFGVARPGTETSDVVCKPCAPGTFSNTTSSTDICRPHQICSVVAIPGNASMDAVCTSTSPTRSMAPGAVHLPQPVSTRSQHTQPTPGPSTAPSTSILLPMGPSPPAEGSTGDGSGEGEGSEGSGLPAQVAFTPYAPEPGSTCRLREYYDQTAQMCCAKCPPGQHAKVFCTKTSDTVCDSCEDSTYTQLWNWVPECLSCSSRCSSDQVETQACTREQNRICTCRPGWYCALSKQEGCRLCAPLSKCRPGFGVARPGTETSDVVCKPCAPGTFSNTTSSTDICRPHQICSVVAIPGNASMDAVCTSTSPTRSMAPGAVHLPQPVSTR

SEQ ID NO: 31 - DNA, 3531 bp, synthetic construct
  misc_feature 1..3531: note = IL-17RA/RC-Fc-TNFR2 (tandem repeat)
  source 1..3531: mol_type = other DNA
atgggtgctgcgcgcagtccaccgagtgctgtgcccggtccattgctgggattgctgctccttcttcttggggtgcttgccccaggtggagcaagccttcggttgctcgaccacagggcccccgtctgctcccaacctggcctgaattgtacagtcaagaactcagactgcttggatgattcatggattcatccacgaaacctcacgcctagcagtcctaaagatttgcaaattcaacttcatttcgcgcacacgcagcaaggagatttggtgcctgttgctcatattgagtggactcttcaaacggacgcctcaattctgtacttggagggagcagaactgtccgttctgcagcttgacacaaacgaaaggctctgtgtcagattcgagttccttagtaaacttcgacatcatcacaggagatggcgatttacattctcccatttcgtggtcgatccgggccaagaatacgaagttacggtgcaccacctgccgaagccaatccccgacggggacccgaaccaccagtccaagaattttctcgttcccgactgtgagcaccctaggatgaaagtgaccacaccttgcatgtcatcagccttgccttggttgaatgtcagcgctgatggagacaatgtgcatctcgtcctgaatgtgtccgaggaacaacattttggactgtctctgtactggaatcaggtacagggcccccctaaaccaaggtggcacaaaaatttgaccggaccgcaaatcatcacactcaatcatactgatcttgtgccttgtctgtgcattcaagtttggccactggagccagactctgtgagaactaatatctgcccttttcgggaggacccgagggcccatcagaatttgtggcaagctgcacgactgcggcttctgacgttgcaatcatggctgcttgacgcgccttgttcccttccagcagaggcagcgctctgctggagggctccaggaggtgacccctgccagccactcgtgccgccactgagttgggaaaatgtcactgtggataaggtccttgagtttccactgctgaagggacatccaaacctttgcgtccaagttaactcttcagagaagcttcagttgcaggagtgtttgtgggcggactctttgggccccctgaaggatgacgtcctccttctcgaaacgcgaggcccacaggataatcgcagcctttgcgcgctggagccaagtggatgcacatcattgccatccaaggcctctacccgggctgctcgactcggggagtatctgctgcaggatctgcagtctggacaatgcctccagctgtgggacgacgatctcggggctctctgggcctgcccaatggacaagtatatccataagaccggtatcgagggcaggatggaccgcaatactgggcggggcggggaggaaaagaaaaaggagaaggaaaaggaggaacaggaggaaagagagactaagaccccagaatgtcccagccatactcagcccctgggggtgttcctgtttccccctaaacctaaggataccctgatgatcagcaggacacccgaggtgacctgcgtggtcgtggatgtgagccaggaagatcccgaagtgcagttcaactggtacgtggatggcgtggaagtgcacaacgccaagaccaagcccagagaagagcagttcaactccacctacagagtggtgagcgtgctgaccgtgctgcaccaggactggctgaacggcaaggagtacaagtgcaaggtgtccaacaaaggcctgcccagctccatcgagaagaccatcagcaaagccaaaggccagcccagagaaccccaggtgtacaccctgcctcccagccaggaagagatgaccaagaaccaggtgtccctgacctgcctggtgaaaggcttctaccccagcgacatcgccgtggagtgggaaagcaacggccagcccgagaacaattacaagacaacccctcccgtgctggatagcgatggcagcttctttctgtacagcagactgaccgtggacaagagcagatggcaggaaggcaacgtgttcagctgcagcgtgatgcacgaagccctgcacaaccactacacccagaagagcctgtccctgagcctgggcaagggtggaggtggttctggaggtggaggatctggaggaggtggttctctcgagctgcccgcccaggtggcttttaccccttacgcccccgagcccggaagcacctgtagactgagagagtactacgaccagactgctcagatgtgctgcgccaaatgccctcctggccagcacgccaaggtgttctgcaccaagacctccgacaccgtctgcgactcctgcgaggattctacctatacccagctgtggaattgggtgcctgagtgcctgtcctgcagctctagatgctcctctgatcaagtggaaacccaggcctgtaccagagagcagaaccggatctgtacatgtcggcctggttggtactgtgctctgtccaagcaagagggctgtcggctgtgcgctcctctgtccaagtgccgccctggcttcggcgtggccagaccaggcaccgagacatctgacgtggtgtgcaagccttgtgccccaggaaccttctccaacaccacctccagcacagatatctgcagacctcaccagatctgctccgtggtcgccatccctggcaacgcctctatggacgcagtttgcacctctacaagccccaccagatccatggctccaggcgccgtgcacctgcctcagcctgtgtccacccggtctcagcacacccagcctacccccggcccctctaccgccccttccacatccatcctgctgcctatgggccctagccctcctgccgaaggctccaccggcgacggtagtggtgagggcgaagggtcagagggatctggactgcccgcccaggtggcttttaccccttacgcccccgagcccggaagcacctgtagactgagagagtactacgaccagactgctcagatgtgctgcgccaaatgccctcctggccagcacgccaaggtgttctgcaccaagacctccgacaccgtctgcgactcctgcgaggattctacctatacccagctgtggaattgggtgcctgagtgcctgtcctgcagctctagatgctcctctgatcaagtggaaacccaggcctgtaccagagagcagaaccggatctgtacatgtcggcctggttggtactgtgctctgtccaagcaagagggctgtcggctgtgcgctcctctgtccaagtgccgccctggcttcggcgtggccagaccaggcaccgagacatctgacgtggtgtgcaagccttgtgccccaggaaccttctccaacaccacctccagcacagatatctgcagacctcaccagatctgctccgtggtcgccatccctggcaacgcctctatggacgcagtttgcacctctacaagccccaccagatccatggctccaggcgccgtgcacctgcctcagcctgtgtccacccggtaa

SEQ ID NO: 32 - protein, 932 aa, synthetic construct
  REGION 1..932: note = IL-17RA/RC-Fc-TNFR2 (T1T4-35)
LRLLDHRAPVCSQPGLNCTVKNSDCLDDSWIHPRNLTPSSPKDLQIQLHFAHTQQGDLVPVAHIEWTLQTDASILYLEGAELSVLQLDTNERLCVRFEFLSKLRHHHRRWRFTFSHFVVDPGQEYEVTVHHLPKPIPDGDPNHQSKNFLVPDCEHPRMKVTTPCMSSALPWLNVSADGDNVHLVLNVSEEQHFGLSLYWNQVQGPPKPRWHKNLTGPQIITLNHTDLVPCLCIQVWPLEPDSVRTNICPFREDPRAHQNLWQAARLRLLTLQSWLLDAPCSLPAEAALCWRAPGGDPCQPLVPPLSWENVTVDKVLEFPLLKGHPNLCVQVNSSEKLQLQECLWADSLGPLKDDVLLLETRGPQDNRSLCALEPSGCTSLPSKASTRAARLGEYLLQDLQSGQCLQLWDDDLGALWACPMDKYIHKTGIEGRMDRNTGRGGEEKKKEKEKEEQEERETKTPECPSHTQPLGVFLFPPKPKDTLMISRTPEVTCVVVDVSQEDPEVQFNWYVDGVEVHNAKTKPREEQFNSTYRVVSVLTVLHQDWLNGKEYKCKVSNKGLPSSIEKTISKAKGQPREPQVYTLPPSQEEMTKNQVSLTCLVKGFYPSDIAVEWESNGQPENNYKTTPPVLDSDGSFFLYSRLTVDKSRWQEGNVFSCSVMHEALHNHYTQKSLSLSLGKGGGGSGGGGSGGGGSLEVPAQVVLTPYKPEPGYECQISQEYYDRKAQMCCAKCPPGQYVKHFCNKTSDTVCADCEASMYTQVWNQFRTCLSCSSSCTTDQVEIRACTKQQNRVCACEAGRYCALKTHSGSCRQCMRLSKCGPGFGVASSRAPNGNVLCKACAPGTFSDTTSSTDVCRPHRICSILAIPGNASTDAVCAPESPTLSAIPRTLYVSQPEPTRSQPLDQEPGPSQTPSILTSLGSTPIIEQSTKGG

SEQ ID NO: 33 - protein, 245 aa, synthetic construct
  REGION 1..245: note = hyFc
RNTGRGGEEKKKEKEKEEQEERETKTPECPSHTQPLGVFLFPPKPKDTLMISRTPEVTCVVVDVSQEDPEVQFNWYVDGVEVHNAKTKPREEQFNSTYRVVSVLTVLHQDWLNGKEYKCKVSNKGLPSSIEKTISKAKGQPREPQVYTLPPSQEEMTKNQVSLTCLVKGFYPSDIAVEWESNGQPENNYKTTPPVLDSDGSFFLYSRLTVDKSRWQEGNVFSCSVMHEALHNHYTQKSLSLSLGK

SEQ ID NO: 34 - protein, 245 aa, synthetic construct
  REGION 1..245: note = hyFC+YTE
RNTGRGGEEKKKEKEKEEQEERETKTPECPSHTQPLGVFLFPPKPKDTLYITREPEVTCVVVDVSQEDPEVQFNWYVDGVEVHNAKTKPREEQFNSTYRVVSVLTVLHQDWLNGKEYKCKVSNKGLPSSIEKTISKAKGQPREPQVYTLPPSQEEMTKNQVSLTCLVKGFYPSDIAVEWESNGQPENNYKTTPPVLDSDGSFFLYSRLTVDKSRWQEGNVFSCSVMHEALHNHYTQKSLSLSLGK

SEQ ID NO: 35 - protein, 245 aa, synthetic construct
  REGION 1..245: note = hyFc1+KF
RNTGRGGEEKKKEKEKEEQEERETKTPECPSHTQPLGVFLFPPKPKDTLMISRTPEVTCVVVDVSQEDPEVQFNWYVDGVEVHNAKTKPREEQFNSTYRVVSVLTVLHQDWLNGKEYKCKVSNKGLPSSIEKTISKAKGQPREPQVYTLPPSQEEMTKNQVSLTCLVKGFYPSDIAVEWESNGQPENNYKTTPPVLDSDGSFFLYSRLTVDKSRWQEGNVFSCSVMHEALKFHYTQKSLSLSLGK

SEQ ID NO: 36 - protein, 245 aa, synthetic construct
  REGION 1..245: note = hyFc1+YTE+KF
RNTGRGGEEKKKEKEKEEQEERETKTPECPSHTQPLGVFLFPPKPKDTLYITREPEVTCVVVDVSQEDPEVQFNWYVDGVEVHNAKTKPREEQFNSTYRVVSVLTVLHQDWLNGKEYKCKVSNKGLPSSIEKTISKAKGQPREPQVYTLPPSQEEMTKNQVSLTCLVKGFYPSDIAVEWESNGQPENNYKTTPPVLDSDGSFFLYSRLTVDKSRWQEGNVFSCSVMHEALKFHYTQKSLSLSLGK

SEQ ID NO: 37 - protein, 245 aa, synthetic construct
  REGION 1..245: note = hyFc1+LS
RNTGRGGEEKKKEKEKEEQEERETKTPECPSHTQPLGVFLFPPKPKDTLMISRTPEVTCVVVDVSQEDPEVQFNWYVDGVEVHNAKTKPREEQFNSTYRVVSVLTVLHQDWLNGKEYKCKVSNKGLPSSIEKTISKAKGQPREPQVYTLPPSQEEMTKNQVSLTCLVKGFYPSDIAVEWESNGQPENNYKTTPPVLDSDGSFFLYSRLTVDKSRWQEGNVFSCSVLHEALHSHYTQKSLSLSLGK

SEQ ID NO: 38 - protein, 245 aa, synthetic construct
  REGION 1..245: note = hyFc1+YTE+LS
RNTGRGGEEKKKEKEKEEQEERETKTPECPSHTQPLGVFLFPPKPKDTLYITREPEVTCVVVDVSQEDPEVQFNWYVDGVEVHNAKTKPREEQFNSTYRVVSVLTVLHQDWLNGKEYKCKVSNKGLPSSIEKTISKAKGQPREPQVYTLPPSQEEMTKNQVSLTCLVKGFYPSDIAVEWESNGQPENNYKTTPPVLDSDGSFFLYSRLTVDKSRWQEGNVFSCSVLHEALHSHYTQKSLSLSLGK

SEQ ID NO: 39 - protein, 245 aa, synthetic construct
  REGION 1..245: note = hyFc GG
RNTGRGGEEKKGGKEKEEQEERETKTPECPSHTQPLGVFLFPPKPKDTLMISRTPEVTCVVVDVSQEDPEVQFNWYVDGVEVHNAKTKPREEQFNSTYRVVSVLTVLHQDWLNGKEYKCKVSNKGLPSSIEKTISKAKGQPREPQVYTLPPSQEEMTKNQVSLTCLVKGFYPSDIAVEWESNGQPENNYKTTPPVLDSDGSFFLYSRLTVDKSRWQEGNVFSCSVMHEALHNHYTQKSLSLSLGK

SEQ ID NO: 40 - protein, 245 aa, synthetic construct
  REGION 1..245: note = hyFc GS
RNTGRGGEEKKGSKEKEEQEERETKTPECPSHTQPLGVFLFPPKPKDTLMISRTPEVTCVVVDVSQEDPEVQFNWYVDGVEVHNAKTKPREEQFNSTYRVVSVLTVLHQDWLNGKEYKCKVSNKGLPSSIEKTISKAKGQPREPQVYTLPPSQEEMTKNQVSLTCLVKGFYPSDIAVEWESNGQPENNYKTTPPVLDSDGSFFLYSRLTVDKSRWQEGNVFSCSVMHEALHNHYTQKSLSLSLGK

SEQ ID NO: 41 - protein, 245 aa, synthetic construct
  REGION 1..245: note = hyFc SG
RNTGRGGEEKKSGKEKEEQEERETKTPECPSHTQPLGVFLFPPKPKDTLMISRTPEVTCVVVDVSQEDPEVQFNWYVDGVEVHNAKTKPREEQFNSTYRVVSVLTVLHQDWLNGKEYKCKVSNKGLPSSIEKTISKAKGQPREPQVYTLPPSQEEMTKNQVSLTCLVKGFYPSDIAVEWESNGQPENNYKTTPPVLDSDGSFFLYSRLTVDKSRWQEGNVFSCSVMHEALHNHYTQKSLSLSLGK

SEQ ID NO: 42 - protein, 245 aa, synthetic construct
  REGION 1..245: note = hyFc SS
RNTGRGGEEKKSSKEKEEQEERETKTPECPSHTQPLGVFLFPPKPKDTLMISRTPEVTCVVVDVSQEDPEVQFNWYVDGVEVHNAKTKPREEQFNSTYRVVSVLTVLHQDWLNGKEYKCKVSNKGLPSSIEKTISKAKGQPREPQVYTLPPSQEEMTKNQVSLTCLVKGFYPSDIAVEWESNGQPENNYKTTPPVLDSDGSFFLYSRLTVDKSRWQEGNVFSCSVMHEALHNHYTQKSLSLSLGK

SEQ ID NO: 43 - protein, 227 aa, synthetic construct
  REGION 1..227: note = Mouse Fc
VPRDCGCKPCICTVPEVSSVFIFPPKPKDVLTITLTPKVTCVVVDISKDDPEVQFSWFVDDVEVHTAQTQPREEQFNSTFRSVSELPIMHQDWLNGKEFKCRVNSAAFPAPIEKTISKTKGRPKAPQVYTIPPPKEQMAKDKVSLTCMITDFFPEDITVEWQWNGQPAENYKNTQPIMNTNGSYFVYSKLNVQKSNWEAGNTFTCSVLHEGLHNHHTEKSLSHSPGK

SEQ ID NO: 44 - protein, 232 aa, synthetic construct
  REGION 1..232: note = IgG1
EPKSCDKTHTCPPCPAPELLGGPSVFLFPPKPKDTLMISRTPEVTCVVVDVSHEDPEVKFNWYVDGVEVHNAKTKPREEQYNSTYRVVSVLTVLHQDWLNGKEYKCKVSNKALPAPIEKTISKAKGQPREPQVYTLPPSRDELTKNQVSLTCLVKGFYPSDIAVEWESNGQPENNYKTTPPVLDSDGSFFLYSKLTVDKSRWQQGNVFSCSVMHEALHNHYTQKSLSLSPGK

SEQ ID NO: 45 - protein, 223 aa, synthetic construct
  REGION 1..223: note = IgG4
THTCPPCPSHTQPLGVFLFPPKPKDTLMISRTPEVTCVVVDVSQEDPEVQFNWYVDGVEVHNAKTKPREEQFNSTYRVVSVLTVLHQDWLNGKEYKCKVSNKGLPSSIEKTISKAKGQPREPQVYTLPPSQEEMTKNQVSLTCLVKGFYPSDIAVEWESNGQPENNYKTTPPVLDSDGSFFLYSRLTVDKSRWQEGNVFSCSVMHEALHNHYTQKSLSLSLGK

SEQ ID NO: 46 - protein, 245 aa, synthetic construct
  REGION 1..245: note = hyFc2(GG)+YTE
RNTGRGGEEKKGGKEKEEQEERETKTPECPSHTQPLGVFLFPPKPKDTLYITREPEVTCVVVDVSQEDPEVQFNWYVDGVEVHNAKTKPREEQFNSTYRVVSVLTVLHQDWLNGKEYKCKVSNKGLPSSIEKTISKAKGQPREPQVYTLPPSQEEMTKNQVSLTCLVKGFYPSDIAVEWESNGQPENNYKTTPPVLDSDGSFFLYSRLTVDKSRWQEGNVFSCSVMHEALHNHYTQKSLSLSLGK

SEQ ID NO: 47 - protein, 245 aa, synthetic construct
  REGION 1..245: note = hyFc2(GG)+KF
RNTGRGGEEKKGGKEKEEQEERETKTPECPSHTQPLGVFLFPPKPKDTLMISRTPEVTCVVVDVSQEDPEVQFNWYVDGVEVHNAKTKPREEQFNSTYRVVSVLTVLHQDWLNGKEYKCKVSNKGLPSSIEKTISKAKGQPREPQVYTLPPSQEEMTKNQVSLTCLVKGFYPSDIAVEWESNGQPENNYKTTPPVLDSDGSFFLYSRLTVDKSRWQEGNVFSCSVMHEALKFHYTQKSLSLSLGK

SEQ ID NO: 48 - protein, 245 aa, synthetic construct
  REGION 1..245: note = hyFc2(GG)+YTE+KF
RNTGRGGEEKKGGKEKEEQEERETKTPECPSHTQPLGVFLFPPKPKDTLYITREPEVTCVVVDVSQEDPEVQFNWYVDGVEVHNAKTKPREEQFNSTYRVVSVLTVLHQDWLNGKEYKCKVSNKGLPSSIEKTISKAKGQPREPQVYTLPPSQEEMTKNQVSLTCLVKGFYPSDIAVEWESNGQPENNYKTTPPVLDSDGSFFLYSRLTVDKSRWQEGNVFSCSVMHEALKFHYTQKSLSLSLGK

SEQ ID NO: 49 - protein, 245 aa, synthetic construct
  REGION 1..245: note = hyFc2(GG)+LS
RNTGRGGEEKKGGKEKEEQEERETKTPECPSHTQPLGVFLFPPKPKDTLMISRTPEVTCVVVDVSQEDPEVQFNWYVDGVEVHNAKTKPREEQFNSTYRVVSVLTVLHQDWLNGKEYKCKVSNKGLPSSIEKTISKAKGQPREPQVYTLPPSQEEMTKNQVSLTCLVKGFYPSDIAVEWESNGQPENNYKTTPPVLDSDGSFFLYSRLTVDKSRWQEGNVFSCSVLHEALHSHYTQKSLSLSLGK

SEQ ID NO: 50 - protein, 245 aa, synthetic construct
  REGION 1..245: note = hyFc2(GG)+YTE+LS
RNTGRGGEEKKGGKEKEEQEERETKTPECPSHTQPLGVFLFPPKPKDTLYITREPEVTCVVVDVSQEDPEVQFNWYVDGVEVHNAKTKPREEQFNSTYRVVSVLTVLHQDWLNGKEYKCKVSNKGLPSSIEKTISKAKGQPREPQVYTLPPSQEEMTKNQVSLTCLVKGFYPSDIAVEWESNGQPENNYKTTPPVLDSDGSFFLYSRLTVDKSRWQEGNVFSCSVLHEALHSHYTQKSLSLSLGK

SEQ ID NO: 51 - protein, 245 aa, synthetic construct
  REGION 1..245: note = hyFc2(GS)+YTE
RNTGRGGEEKKGSKEKEEQEERETKTPECPSHTQPLGVFLFPPKPKDTLYITREPEVTCVVVDVSQEDPEVQFNWYVDGVEVHNAKTKPREEQFNSTYRVVSVLTVLHQDWLNGKEYKCKVSNKGLPSSIEKTISKAKGQPREPQVYTLPPSQEEMTKNQVSLTCLVKGFYPSDIAVEWESNGQPENNYKTTPPVLDSDGSFFLYSRLTVDKSRWQEGNVFSCSVMHEALHNHYTQKSLSLSLGK

SEQ ID NO: 52 - protein, 245 aa, synthetic construct
  REGION 1..245: note = hyFc2(GS)+KF
RNTGRGGEEKKGSKEKEEQEERETKTPECPSHTQPLGVFLFPPKPKDTLMISRTPEVTCVVVDVSQEDPEVQFNWYVDGVEVHNAKTKPREEQFNSTYRVVSVLTVLHQDWLNGKEYKCKVSNKGLPSSIEKTISKAKGQPREPQVYTLPPSQEEMTKNQVSLTCLVKGFYPSDIAVEWESNGQPENNYKTTPPVLDSDGSFFLYSRLTVDKSRWQEGNVFSCSVMHEALKFHYTQKSLSLSLGK

SEQ ID NO: 53 - protein, 245 aa, synthetic construct
  REGION 1..245: note = hyFc2(GS)+YTE+KF
RNTGRGGEEKKGSKEKEEQEERETKTPECPSHTQPLGVFLFPPKPKDTLYITREPEVTCVVVDVSQEDPEVQFNWYVDGVEVHNAKTKPREEQFNSTYRVVSVLTVLHQDWLNGKEYKCKVSNKGLPSSIEKTISKAKGQPREPQVYTLPPSQEEMTKNQVSLTCLVKGFYPSDIAVEWESNGQPENNYKTTPPVLDSDGSFFLYSRLTVDKSRWQEGNVFSCSVMHEALKFHYTQKSLSLSLGK

SEQ ID NO: 54 - protein, 245 aa, synthetic construct
  REGION 1..245: note = hyFc2(GS)+LS
RNTGRGGEEKKGSKEKEEQEERETKTPECPSHTQPLGVFLFPPKPKDTLMISRTPEVTCVVVDVSQEDPEVQFNWYVDGVEVHNAKTKPREEQFNSTYRVVSVLTVLHQDWLNGKEYKCKVSNKGLPSSIEKTISKAKGQPREPQVYTLPPSQEEMTKNQVSLTCLVKGFYPSDIAVEWESNGQPENNYKTTPPVLDSDGSFFLYSRLTVDKSRWQEGNVFSCSVLHEALHSHYTQKSLSLSLGK

SEQ ID NO: 55 - protein, 245 aa, synthetic construct
  REGION 1..245: note = hyFc2(GS)+YTE+LS
RNTGRGGEEKKGSKEKEEQEERETKTPECPSHTQPLGVFLFPPKPKDTLYITREPEVTCVVVDVSQEDPEVQFNWYVDGVEVHNAKTKPREEQFNSTYRVVSVLTVLHQDWLNGKEYKCKVSNKGLPSSIEKTISKAKGQPREPQVYTLPPSQEEMTKNQVSLTCLVKGFYPSDIAVEWESNGQPENNYKTTPPVLDSDGSFFLYSRLTVDKSRWQEGNVFSCSVLHEALHSHYTQKSLSLSLGK

SEQ ID NO: 56 - protein, 245 aa, synthetic construct
  REGION 1..245: note = hyFc2(SG)+YTE
RNTGRGGEEKKSGKEKEEQEERETKTPECPSHTQPLGVFLFPPKPKDTLYITREPEVTCVVVDVSQEDPEVQFNWYVDGVEVHNAKTKPREEQFNSTYRVVSVLTVLHQDWLNGKEYKCKVSNKGLPSSIEKTISKAKGQPREPQVYTLPPSQEEMTKNQVSLTCLVKGFYPSDIAVEWESNGQPENNYKTTPPVLDSDGSFFLYSRLTVDKSRWQEGNVFSCSVMHEALHNHYTQKSLSLSLGK

SEQ ID NO: 57 - protein, 245 aa, synthetic construct
  REGION 1..245: note = hyFc2(SG)+KF
RNTGRGGEEKKSGKEKEEQEERETKTPECPSHTQPLGVFLFPPKPKDTLMISRTPEVTCVVVDVSQEDPEVQFNWYVDGVEVHNAKTKPREEQFNSTYRVVSVLTVLHQDWLNGKEYKCKVSNKGLPSSIEKTISKAKGQPREPQVYTLPPSQEEMTKNQVSLTCLVKGFYPSDIAVEWESNGQPENNYKTTPPVLDSDGSFFLYSRLTVDKSRWQEGNVFSCSVMHEALKFHYTQKSLSLSLGK

SEQ ID NO: 58 - protein, 245 aa, synthetic construct
  REGION 1..245: note = hyFc2(SG)+YTE+KF
RNTGRGGEEKKSGKEKEEQEERETKTPECPSHTQPLGVFLFPPKPKDTLYITREPEVTCVVVDVSQEDPEVQFNWYVDGVEVHNAKTKPREEQFNSTYRVVSVLTVLHQDWLNGKEYKCKVSNKGLPSSIEKTISKAKGQPREPQVYTLPPSQEEMTKNQVSLTCLVKGFYPSDIAVEWESNGQPENNYKTTPPVLDSDGSFFLYSRLTVDKSRWQEGNVFSCSVMHEALKFHYTQKSLSLSLGK

SEQ ID NO: 59 - protein, 245 aa, synthetic construct
  REGION 1..245: note = hyFc2(SG)+LS
RNTGRGGEEKKSGKEKEEQEERETKTPECPSHTQPLGVFLFPPKPKDTLMISRTPEVTCVVVDVSQEDPEVQFNWYVDGVEVHNAKTKPREEQFNSTYRVVSVLTVLHQDWLNGKEYKCKVSNKGLPSSIEKTISKAKGQPREPQVYTLPPSQEEMTKNQVSLTCLVKGFYPSDIAVEWESNGQPENNYKTTPPVLDSDGSFFLYSRLTVDKSRWQEGNVFSCSVLHEALHSHYTQKSLSLSLGK

SEQ ID NO: 60 - protein, 245 aa, synthetic construct
  REGION 1..245: note = hyFc2(SG)+YTE+LS
RNTGRGGEEKKSGKEKEEQEERETKTPECPSHTQPLGVFLFPPKPKDTLYITREPEVTCVVVDVSQEDPEVQFNWYVDGVEVHNAKTKPREEQFNSTYRVVSVLTVLHQDWLNGKEYKCKVSNKGLPSSIEKTISKAKGQPREPQVYTLPPSQEEMTKNQVSLTCLVKGFYPSDIAVEWESNGQPENNYKTTPPVLDSDGSFFLYSRLTVDKSRWQEGNVFSCSVLHEALHSHYTQKSLSLSLGK

SEQ ID NO: 61 - protein, 245 aa, synthetic construct
  REGION 1..245: note = hyFc2(SS)+YTE
RNTGRGGEEKKSSKEKEEQEERETKTPECPSHTQPLGVFLFPPKPKDTLYITREPEVTCVVVDVSQEDPEVQFNWYVDGVEVHNAKTKPREEQFNSTYRVVSVLTVLHQDWLNGKEYKCKVSNKGLPSSIEKTISKAKGQPREPQVYTLPPSQEEMTKNQVSLTCLVKGFYPSDIAVEWESNGQPENNYKTTPPVLDSDGSFFLYSRLTVDKSRWQEGNVFSCSVMHEALHNHYTQKSLSLSLGK

SEQ ID NO: 62 - protein, 245 aa, synthetic construct
  REGION 1..245: note = hyFc2(SS)+KF
RNTGRGGEEKKSSKEKEEQEERETKTPECPSHTQPLGVFLFPPKPKDTLMISRTPEVTCVVVDVSQEDPEVQFNWYVDGVEVHNAKTKPREEQFNSTYRVVSVLTVLHQDWLNGKEYKCKVSNKGLPSSIEKTISKAKGQPREPQVYTLPPSQEEMTKNQVSLTCLVKGFYPSDIAVEWESNGQPENNYKTTPPVLDSDGSFFLYSRLTVDKSRWQEGNVFSCSVMHEALKFHYTQKSLSLSLGK

SEQ ID NO: 63 - protein, 245 aa, synthetic construct
  REGION 1..245: note = hyFc2(SS)+YTE+KF
RNTGRGGEEKKSSKEKEEQEERETKTPECPSHTQPLGVFLFPPKPKDTLYITREPEVTCVVVDVSQEDPEVQFNWYVDGVEVHNAKTKPREEQFNSTYRVVSVLTVLHQDWLNGKEYKCKVSNKGLPSSIEKTISKAKGQPREPQVYTLPPSQEEMTKNQVSLTCLVKGFYPSDIAVEWESNGQPENNYKTTPPVLDSDGSFFLYSRLTVDKSRWQEGNVFSCSVMHEALKFHYTQKSLSLSLGK

SEQ ID NO: 64 - protein, 245 aa, synthetic construct
  REGION 1..245: note = hyFc2(SS)+LS
RNTGRGGEEKKSSKEKEEQEERETKTPECPSHTQPLGVFLFPPKPKDTLMISRTPEVTCVVVDVSQEDPEVQFNWYVDGVEVHNAKTKPREEQFNSTYRVVSVLTVLHQDWLNGKEYKCKVSNKGLPSSIEKTISKAKGQPREPQVYTLPPSQEEMTKNQVSLTCLVKGFYPSDIAVEWESNGQPENNYKTTPPVLDSDGSFFLYSRLTVDKSRWQEGNVFSCSVLHEALHSHYTQKSLSLSLGK

SEQ ID NO: 65 - protein, 245 aa, synthetic construct
  REGION 1..245: note = hyFc2(SS)+YTE+LS
RNTGRGGEEKKSSKEKEEQEERETKTPECPSHTQPLGVFLFPPKPKDTLYITREPEVTCVVVDVSQEDPEVQFNWYVDGVEVHNAKTKPREEQFNSTYRVVSVLTVLHQDWLNGKEYKCKVSNKGLPSSIEKTISKAKGQPREPQVYTLPPSQEEMTKNQVSLTCLVKGFYPSDIAVEWESNGQPENNYKTTPPVLDSDGSFFLYSRLTVDKSRWQEGNVFSCSVLHEALHSHYTQKSLSLSLGK

SEQ ID NO: 66 - protein, 460 aa, synthetic construct
  REGION 1..460: note = T1Rf
MGAARSPPSAVPGPLLGLLLLLLGVLAPGGASLRLLDHRALVCSQPGLNCTVKNSTCLDDSWIHPRNLTPSSPKDLQIQLHFAHTQQGDLFPVAHIEWTLQTDASILYLEGAELSVLQLNTNERLCVRFEFLSKLRHHAAAARWRFTFSHFVVDPDQEYEVTVHHLPKPIPDGDPNHQSKNFLVPDCEHARMKVTTPCMSSALPWLNVSADGDNVHLVLNVSEEQHFGLSLYWNQVQGPPKPRWHKNLTGPQIITLNHTDLVPCLCIQVWPLEPDSVRTNICPFREDPRAHQNLWQAARLQLLTLQSWLLDAPCSLPAEAALCWRAPGGDPCQPLVPPLSWENVTVDKVLEFPLLKGHPNLCVQVNSSEKLQLQECLWADSLGPLKDDVLLLETRGPQDNRSLCALEPSGCTSLPSKASTRAARLGEYLLQDLQSGQCLQLWDDDLGALWACPMDKYIHK

SEQ ID NO: 67 - protein, 458 aa, synthetic construct
  REGION 1..458: note = T1a
MGAARSPPSAVPGPLLGLLLLLLGVLAPGGASLRLLDHRAPVCSQPGLNCTVKNSDCLDDSWIHPRNLTPSSPKDLQIQLHFAHTQQGDLVPVAHIEWTLQTDASILYLEGAELSVLQLDTNERLCVRFEFLSKLRHHHRRWRFTFSHFVVDPGQEYEVTVHHLPKPIPDGDPNHQSKNFLVPDCEHARMKVTTPCMSSALPWLNVSADGDNVHLVLNVSEEQHFGLSLYWNQVQGPPKPRWHKNLTGPQIITLNHTDLVPCLCIQVWPLEPDSVRTNICPFREDPRAHQNLWQAARLRLLTLQSWLLDAPCSLPAEAALCWRAPGGDPCQPLVPPLSWENVTVDKVLEFPLLKGHPNLCVQVNSSEKLQLQECLWADSLGPLKDDVLLLETRGPQDNRSLCALEPSGCTSLPSKASTRAARLGEYLLQDLQSGQCLQLWDDDLGALWACPMDKYIHK

SEQ ID NO: 68 - protein, 458 aa, synthetic construct
  REGION 1..458: note = T1b
MGAARSPPSAVPGPLLGLLLLLLGVLAPGGASLRLLDHRAPVCSQPGLNCTVKNSDCLDDSWIHPRNLTPSSPKDLQIQLHFAHTQQGDLVPVAHIEWTLQTDASILYLEGAELSVLQLDTNERLCVRFEFLSKLRHHHRRWRFTFSHFVVDPGQEYEVTVHHLPKPIPDGDPNHQSKNFLVPDCEHPRMKVTTPCMSSALPWLNVSADGDNVHLVLNVSEEQHFGLSLYWNQVQGPPKPRWHKNLTGPQIITLNHTDLVPCLCIQVWPLEPDSVRTNICPFREDPRAHQNLWQAARLRLLTLQSWLLDAPCSLPAEAALCWRAPGGDPCQPLVPPLSWENVTVDKVLEFPLLKGHPNLCVQVNSSEKLQLQECLWADSLGPLKDDVLLLETRGPQDNRSLCALEPSGCTSLPSKASTRAARLGEYLLQDLQSGQCLQLWDDDLGALWACPMDKYIHK

SEQ ID NO: 69 - protein, 458 aa, synthetic construct; identical to SEQ ID NO: 68
  REGION 1..458: note = T1c

SEQ ID NO: 70 - protein, 235 aa, synthetic construct
  REGION 1..235: note = T4 wt (wt TNFR2)
LPAQVAFTPYAPEPGSTCRLREYYDQTAQMCCSKCSPGQHAKVFCTKTSDTVCDSCEDSTYTQLWNWVPECLSCGSRCSSDQVETQACTREQNRICTCRPGWYCALSKQEGCRLCAPLRKCRPGFGVARPGTETSDVVCKPCAPGTFSNTTSSTDICRPHQICNVVAIPGNASMDAVCTSTSPTRSMAPGAVHLPQPVSTRSQHTQPTPEPSTAPSTSFLLPMGPSPPAEGSTGD

SEQ ID NO: 71 - protein, 235 aa, synthetic construct
  REGION 1..235: note = T4a
LPAQVAFTPYAPEPGSTCRLREYYDQTAQMCCAKCSPGQHAKVFCTKTSDTVCDSCEDSTYTQLWNWVPECLSCGSRCSSDQVETQACTREQNRICTCRPGWYCALSKQEGCRLCAPLRKCRPGFGVARPGTETSDVVCKPCAPGTFSNTTSSTDICRPHQICNVVAIPGNASMDAVCTSTSPTRSMAPGAVHLPQPVSTRSQHTQPTPEPSTAPSTSFLLPMGPSPPAEGSTGD

SEQ ID NO: 72 - protein, 235 aa, synthetic construct
  REGION 1..235: note = T4b
LPAQVAFTPYAPEPGSTCRLREYYDQTAQMCCAKCPPGQHAKVFCTKTSDTVCDSCEDSTYTQLWNWVPECLSCGSRCSSDQVETQACTREQNRICTCRPGWYCALSKQEGCRLCAPLRKCRPGFGVARPGTETSDVVCKPCAPGTFSNTTSSTDICRPHQICNVVAIPGNASMDAVCTSTSPTRSMAPGAVHLPQPVSTRSQHTQPTPEPSTAPSTSFLLPMGPSPPAEGSTGD

SEQ ID NO: 73 - protein, 235 aa, synthetic construct
  REGION 1..235: note = T4c
LPAQVAFTPYAPEPGSTCRLREYYDQTAQMCCAKCPPGQHAKVFCTKTSDTVCDSCEDSTYTQLWNWVPECLSCGSRCSSDQVETQACTREQNRICTCRPGWYCALSKQEGCRLCAPLSKCRPGFGVARPGTETSDVVCKPCAPGTFSNTTSSTDICRPHQICNVVAIPGNASMDAVCTSTSPTRSMAPGAVHLPQPVSTRSQHTQPTPEPSTAPSTSFLLPMGPSPPAEGSTGD

SEQ ID NO: 74 - protein, 235 aa, synthetic construct
  REGION 1..235: note = T4d
LPAQVAFTPYAPEPGSTCRLREYYDQTAQMCCAKCPPGQHAKVFCTKTSDTVCDSCEDSTYTQLWNWVPECLSCGSRCSSDQVETQACTREQNRICTCRPGWYCALSKQEGCRLCAPLSKCRPGFGVARPGTETSDVVCKPCAPGTFSNTTSSTDICRPHQICSVVAIPGNASMDAVCTSTSPTRSMAPGAVHLPQPVSTRSQHTQPTPEPSTAPSTSFLLPMGPSPPAEGSTGD

SEQ ID NO: 75 - protein, 235 aa, synthetic construct
  REGION 1..235: note = T4e
LPAQVAFTPYAPEPGSTCRLREYYDQTAQMCCAKCPPGQHAKVFCTKTSDTVCDSCEDSTYTQLWNWVPECLSCGSRCSSDQVETQACTREQNRICTCRPGWYCALSKQEGCRLCAPLSKCRPGFGVARPGTETSDVVCKPCAPGTFSNTTSSTDICRPHQICSVVAIPGNASMDAVCTSTSPTRSMAPGAVHLPQPVSTRSQHTQPTPGPSTAPSTSFLLPMGPSPPAEGSTGD

SEQ ID NO: 76 - protein, 235 aa, synthetic construct
  REGION 1..235: note = T4f
LPAQVAFTPYAPEPGSTCRLREYYDQTAQMCCAKCPPGQHAKVFCTKTSDTVCDSCEDSTYTQLWNWVPECLSCSSRCSSDQVETQACTREQNRICTCRPGWYCALSKQEGCRLCAPLSKCRPGFGVARPGTETSDVVCKPCAPGTFSNTTSSTDICRPHQICSVVAIPGNASMDAVCTSTSPTRSMAPGAVHLPQPVSTRSQHTQPTPEPSTAPSTSFLLPMGPSPPAEGSTGD

SEQ ID NO: 77 - protein, 235 aa, synthetic construct
  REGION 1..235: note = T4g
LPAQVAFTPYAPEPGSTCRLREYYDQTAQMCCAKCPPGQHAKVFCTKTSDTVCDSCEDSTYTQLWNWVPECLSCGSRCSSDQVETQACTREQNRICTCRPGWYCALSKQEGCRLCAPLSKCRPGFGVARPGTETSDVVCKPCAPGTFSNTTSSTDICRPHQICSVVAIPGNASMDAVCTSTSPTRSMAPGAVHLPQPVSTRSQHTQPTPGPSTAPSTSILLPMGPSPPAEGSTGD

SEQ ID NO: 78 - protein, 235 aa, synthetic construct
  REGION 1..235: note = T4h
LPAQVAFTPYAPEPGSTCRLREYYDQTAQMCCAKCPPGQHAKVFCTKTSDTVCDSCEDSTYTQLWNWVPECLSCSSRCSSDQVETQACTREQNRICTCRPGWYCALSKQEGCRLCAPLSKCRPGFGVARPGTETSDVVCKPCAPGTFSNTTSSTDICRPHQICSVVAIPGNASMDAVCTSTSPTRSMAPGAVHLPQPVSTRSQHTQPTPGPSTAPSTSILLPMGPSPPAEGSTGD

SEQ ID NO: 79 - protein, 235 aa, synthetic construct
  REGION 1..235: note = T4i
LPAQVAFTPYAPEPGSTCRLREYYDQTAQMCCSKCSPGQHAKVFCTKTSDTVCDSCEDSTYTQLWNWVPECLSCSSRCSSDQVETQACTREQNRICTCRPGWYCALSKQEGCRLCAPLRKCRPGFGVARPGTETSDVVCKPCAPGTFSNTTSSTDICRPHQICNVVAIPGNASMDAVCTSTSPTRSMAPGAVHLPQPVSTRSQHTQPTPEPSTAPSTSFLLPMGPSPPAEGSTGD

SEQ ID NO: 80 - protein, 448 aa, synthetic construct
  REGION 1..448: note = T4TR
LPAQVAFTPYAPEPGSTCRLREYYDQTAQMCCAKCPPGQHAKVFCTKTSDTVCDSCEDSTYTQLWNWVPECLSCSSRCSSDQVETQACTREQNRICTCRPGWYCALSKQEGCRLCAPLSKCRPGFGVARPGTETSDVVCKPCAPGTFSNTTSSTDICRPHQICSVVAIPGNASMDAVCTSTSPTRSMAPGAVHLPQPVSTRSQHTQPTPGPSTAPSTSILLPMGPSPPAEGSTGDGSGEGEGSEGSGLPAQVAFTPYAPEPGSTCRLREYYDQTAQMCCAKCPPGQHAKVFCTKTSDTVCDSCEDSTYTQLWNWVPECLSCSSRCSSDQVETQACTREQNRICTCRPGWYCALSKQEGCRLCAPLSKCRPGFGVARPGTETSDVVCKPCAPGTFSNTTSSTDICRPHQICSVVAIPGNASMDAVCTSTSPTRSMAPGAVHLPQPVSTR

SEQ ID NO: 81 - protein, 236 aa, synthetic construct
  REGION 1..236: note = T42m
VPAQVVLTPYKPEPGYECQISQEYYDRKAQMCCAKCPPGQYVKHFCNKTSDTVCADCEASMYTQVWNQFRTCLSCSSSCTTDQVEIRACTKQQNRVCACEAGRYCALKTHSGSCRQCMRLSKCGPGFGVASSRAPNGNVLCKACAPGTFSDTTSSTDVCRPHRICSILAIPGNASTDAVCAPESPTLSAIPRTLYVSQPEPTRSQPLDQEPGPSQTPSILTSLGSTPIIEQSTKGG

SEQ ID NO: 82 - protein, 666 aa, synthetic construct
  REGION 1..666: note = tmTNF-alpha
ATGAGCACTGAAAGCATGATCCGGGACGTGGAGCTGGCCGAGGAGGCGCTCCCCAAGAAGACAGGGGGGCCCCAGGGCTCCAGGCGGTGCTTGTTCCTCAGCCTCTTCTCCTTCCTGATCGTGGCAGGCGCCACCACGCTCTTCTGCCTGCTGCACTTTGGAGTGATCGGCCCCCAGAGGGAAGAGTTCCCCAGGGACCTCTCTCTAATCAGCCCTCTGGCCCAGGCAGTAGCCCATGTTGTAGCAAACCCTCAAGCTGAGGGGCAGCTCCAGTGGCTGAACCGCCGGGCCAATGCCCTCCTGGCCAATGGCGTGGAGCTGAGAGATAACCAGCTGGTGGTGCCATCAGAGGGCCTGTACCTCATCTACTCCCAGGTCCTCTTCAAGGGCCAAGGCTGCCCCTCCACCCATGTGCTCCTCACCCACACCATCAGCCGCATCGCCGTCTCCTACCAGACCAAGGTCAACCTCCTCTCTGCCATCAAGAGCCCCTGCCAGAGGGAGACCCCAGAGGGGGCTGAGGCCAAGCCCTGGTATGAGCCCATCTATCTGGGAGGGGTCTTCCAGCTGGAGAAGGGTGACCGACTCAGCGCTGAGATCAATCGGCCCGACTATCTCGACTTTGCCGAGTCTGGGCAGGTCTACTTTGGGATCATTGCCCTGTGA

SEQ ID NO: 83 - protein, 33 aa, synthetic construct
  REGION 1..33: note = linker peptide
GGGGSGGGGSGGGGSEKEKEEQEERTHTCPPCP

SEQ ID NO: 84 - protein, 30 aa, synthetic construct
  REGION 1..30: note = linker peptide
RNTGRGGEEKKGSKEKEEQEERETKTPECP

SEQ ID NO: 85 - protein, 31 aa, synthetic construct
  REGION 1..31: note = linker peptide
RNTGRGGEEKKSGKEKEEQEERETKTPECPP

SEQ ID NO: 86 - protein, 30 aa, synthetic construct
  REGION 1..30: note = linker peptide
RNTGRGGEEKKGGKEKEEQEERETKTPECP

SEQ ID NO: 87 - protein, 30 aa, synthetic construct
  REGION 1..30: note = linker peptide
RNTGRGGEEKKSSKEKEEQEERETKTPECP

SEQ ID NO: 88 - protein, 30 aa, synthetic construct
  REGION 1..30: note = linker peptide
RNTGRGGEEKKKEKEKEEQEERETKTPECP

SEQ ID NO: 89 - protein, 17 aa, synthetic construct
  REGION 1..17: note = linker peptide
GGGGSGGGGSGGGGSLE

SEQ ID NO: 90 - protein, 8 aa, synthetic construct
  REGION 1..8: note = linker peptide
TGIEGRMD

SEQ ID NO: 91 - protein, 23 aa, synthetic construct
  REGION 1..23: note = linker peptide
TGKLSGSASAPKLEEGEFSEARV

SEQ ID NO: 92 - protein, 23 aa, synthetic construct
  REGION 1..23: note = linker peptide
KLSGSASAPKLEEGEFSEARVLE

SEQ ID NO: 93 - protein, 14 aa, synthetic construct
  REGION 1..14: note = linker peptide
TGGSGEGEGSEGSG

SEQ ID NO: 94 - protein, 14 aa, synthetic construct
  REGION 1..14: note = linker peptide
GSGEGEGSEGSGLE

SEQ ID NO: 95 - protein, 13 aa, synthetic construct
  REGION 1..13: note = linker peptide
AEAAAKEAAAAKA

SEQ ID NO: 96 - protein, 15 aa, synthetic construct
  REGION 1..15: note = linker peptide
GGGGSGGGGSGGGGS

SEQ ID NO: 97 - protein, 46 aa, synthetic construct
  REGION 1..46: note = linker peptide
AEAAAKEAAAKEAAAKEAAAKALEAEAAAKEAAAKEAAAKEAAAKA

SEQ ID NO: 98 - protein, 15 aa, synthetic construct
  REGION 1..15: note = linker peptide
EPKSSDKTHTCPPCP

SEQ ID NO: 99 - protein, 15 aa, synthetic construct
  REGION 1..15: note = linker peptide
EPKSCDKTHTCPPCP

SEQ ID NO: 100 - DNA, 20 bp, synthetic construct
  misc_feature 1..20: note = hGAPDH F
  source 1..20: mol_type = other DNA
tcaccagggctgcttttaac

SEQ ID NO: 101 - DNA, 20 bp, synthetic construct
  misc_feature 1..20: note = hGAPDH R
  source 1..20: mol_type = other DNA
gacaagcttcccgttctcag

SEQ ID NO: 102 - DNA, 20 bp, synthetic construct
  misc_feature 1..20: note = hCXCL8 F
  source 1..20: mol_type = other DNA
agctctgtgtgaaggtgcag

SEQ ID NO: 103 - DNA, 23 bp, synthetic construct
  misc_feature 1..23: note = hCXCL8 R
  source 1..23: mol_type = other DNA
tctcagccctcttcaaaaacttc

SEQ ID NO: 104 - DNA, 20 bp, synthetic construct
  misc_feature 1..20: note = hS100A7 F
  source 1..20: mol_type = other DNA
cttccccaacttccttagtg

SEQ ID NO: 105 - DNA, 20 bp, synthetic construct
  misc_feature 1..20: note = hS100A7 R
  source 1..20: mol_type = other DNA
gtagtctgtggctatgtctc

SEQ ID NO: 106 - DNA, 20 bp, synthetic construct
  misc_feature 1..20: note = hCCL20 F
  source 1..20: mol_type = other DNA
gcaagcaactttgactgctg

SEQ ID NO: 107 - DNA, 20 bp, synthetic construct
  misc_feature 1..20: note = hCCL20 R
  source 1..20: mol_type = other DNA
caagtccagtgaggcacaaa

SEQ ID NO: 108 - DNA, 19 bp, synthetic construct
  misc_feature 1..19: note = hBD2 F
  source 1..19: mol_type = other DNA
atcagccatgagggtcttg

SEQ ID NO: 109 - DNA, 18 bp, synthetic construct
  misc_feature 1..18: note = hBD2 R
  source 1..18: mol_type = other DNA
gcagcattttgttccagg

SEQ ID NO: 110 - DNA, 17 bp, synthetic construct
  misc_feature 1..17: note = hLCN2 F
  source 1..17: mol_type = other DNA
tgagtgcacaggtgccg

SEQ ID NO: 111 - DNA, 20 bp, synthetic construct
  misc_feature 1..20: note = hLCN2 R
  source 1..20: mol_type = other DNA
tttagcagacaaggtggggc

SEQ ID NO: 112 - DNA, 20 bp, synthetic construct
  misc_feature 1..20: note = hIL-36 gamma F
  source 1..20: mol_type = other DNA
tttagcagacaaggtggggc

SEQ ID NO: 113 - DNA, 20 bp, synthetic construct
  misc_feature 1..20: note = hIL-36 gamma R
  source 1..20: mol_type = other DNA
aggaggcaatgaaccagtcc

SEQ ID NO: 114 - protein, 288 aa, synthetic construct
  REGION 1..288: note = wtIL-17RA ECD
LRLLDHRALVCSQPGLNCTVKNSTCLDDSWIHPRNLTPSSPKDLQIQLHFAHTQQGDLFPVAHIEWTLQTDASILYLEGAELSVLQLNTNERLCVRFEFLSKLRHHHRRWRFTFSHFVVDPDQEYEVTVHHLPKPIPDGDPNHQSKNFLVPDCEHARMKVTTPCMSSGSLWDPNITVETLEAHQLRVSFTLWNESTHYQILLTSFPHMENHSCFEHMHHIPAPRPEEFHQRSNVTLTLRNLKGCCRHQVQIQPFFSSCLNDCLRHSATVSCPEMPDTPEPIPDYMPLW

SEQ ID NO: 115 - protein, 518 aa, synthetic construct
  REGION 1..518: note = wtIL-17RC ECD
LERLVGPQDATHCSPVSLEPWGDEERLRVQFLAQQSLSLAPVTAATARTALSGLSGADGRREERGRGKSWVCLSLGGSGNTEPQKKGLSCRLWDSDILCLPGDIVPAPGPVLAPTHLQTELVLRCQKETDCDLCLRVAVHLAVHGHWEEPEDEEKFGGAADSGVEEPRNASLQAQVVLSFQAYPTARCVLLEVQVPAALVQFGQSVGSVVYDCFEAALGSEVRIWSYTQPRYEKELNHTQQLPDCRGLEVWNSIPSCWALPWLNVSADGDNVHLVLNVSEEQHFGLSLYWNQVQGPPKPRWHKNLTGPQIITLNHTDLVPCLCIQVWPLEPDSVRTNICPFREDPRAHQNLWQAARLQLLTLQSWLLDAPCSLPAEAALCWRAPGGDPCQPLVPPLSWENVTVDKVLEFPLLKGHPNLCVQVNSSEKLQLQECLWADSLGPLKDDVLLLETRGPQDNRSLCALEPSGCTSLPSKASTRAARLGEYLLQDLQSGQCLQLWDDDLGALWACPMDKYIHKR